European Patent Specification EP 3 696 277 B1, published January 25, 2023. Title: QUANTITATIVE DNA-BASED IMAGING AND SUPER-RESOLUTION IMAGING. Applicant: PRESIDENT AND FELLOWS OF HARVARD COLLEGE. Application TBD. The sequence listing filed with the application follows.

SEQUENCE LISTING (913 sequences)

SEQ ID NO: 1 - DNA, 32 bp, Artificial
  Synthetic Polynucleotide
aggccacctcaccagttcaacagtggcgtttt

SEQ ID NO: 2 - DNA, 32 bp, Artificial
  Synthetic Polynucleotide
cgtcaaagggcgaaaacattctggccatccac

SEQ ID NO: 3 - DNA, 48 bp, Artificial
  Synthetic Polynucleotide
agaatgcgcagcgcagtacttatagctcacacattcaacttcataacc

SEQ ID NO: 4 - DNA, 32 bp, Artificial
  Synthetic Polynucleotide
ccttacacagcaaatcgtttgggtggtaaaac

SEQ ID NO: 5 - DNA, 40 bp, Artificial
  Synthetic Polynucleotide
aattcgcgtctggcctagctttcacaggtcagtaccttta

SEQ ID NO: 6 - DNA, 48 bp, Artificial
  Synthetic Polynucleotide
tggcagatgagtaaaaaatcgccatatttaactgtaatttaggacaac

SEQ ID NO: 7 - DNA, 48 bp, Artificial
  Synthetic Polynucleotide
cacgctggttaaacgggtaaacaatttgggaaggcttgcacatcggaa

SEQ ID NO: 8 - DNA, 32 bp, Artificial
  Synthetic Polynucleotide
acgggcaacagctgggtttctgccagcactca

SEQ ID NO: 9 - DNA, 29 bp, Artificial
  Synthetic Polynucleotide
gacgatcgcgggcctgggaagaaaaatct

SEQ ID NO: 10 - DNA, 48 bp, Artificial
  Synthetic Polynucleotide
gtctgaaaaacaggaagaaggcttcgggtaggaatcattaccgcgccc

SEQ ID NO: 11 - DNA, 40 bp, Artificial
  Synthetic Polynucleotide
aagagacagagatagagacctgaaaaatcaagctattttg

SEQ ID NO: 12 - DNA, 31 bp, Artificial
  Synthetic Polynucleotide
gtttgatgaatcggcaaaatttgcgtattgg

SEQ ID NO: 13 - DNA, 48 bp, Artificial
  Synthetic Polynucleotide
ttttcacccctaaaacaaagaataagcaccattacagcgtcagactgt

SEQ ID NO: 14 - DNA, 40 bp, Artificial
  Synthetic Polynucleotide
ggcatcagggaggtgtcgaggcatatagcgagaggcttat

SEQ ID NO: 15 - DNA, 48 bp, Artificial
  Synthetic Polynucleotide
ttaaatgtcaacccgtcggcgcataaattattctccgtggcggattga

SEQ ID NO: 16 - DNA, 48 bp, Artificial
  Synthetic Polynucleotide
atcacccagccattgctggattatgaacgcgaagggcttagaacaaag

SEQ ID NO: 17 - DNA, 44 bp, Artificial
  Synthetic Polynucleotide
accttctaccctactgcgggatcttaccagtataaagaaaaagc

SEQ ID NO: 18 - DNA, 32 bp, Artificial
  Synthetic Polynucleotide
gagtgttgttctccgagtggtcagtttggaac

SEQ ID NO: 19 - DNA, 40 bp, Artificial
  Synthetic Polynucleotide
gcgccagggtggtcgtgaggcgaagaattatgttcaacag

SEQ ID NO: 20 - DNA, 40 bp, Artificial
  Synthetic Polynucleotide
atcccacggcagcaaccgcaagaaatgacttgtagaacgt

SEQ ID NO: 21 - DNA, 32 bp, Artificial
  Synthetic Polynucleotide
agaatacgagcgtaaatcgtcgctattaatta

SEQ ID NO: 22 - DNA, 32 bp, Artificial
  Synthetic Polynucleotide
ccctcggccaacgcgcaactaaagtaataatt

SEQ ID NO: 23 - DNA, 40 bp, Artificial
  Synthetic Polynucleotide
tatgagcatcagcggggcgctttctaaccgtgcatctgcc

SEQ ID NO: 24 - DNA, 48 bp, Artificial
  Synthetic Polynucleotide
atcggccttgctggtacaatattatcaataatatccggtattctccca

SEQ ID NO: 25 - DNA, 48 bp, Artificial
  Synthetic Polynucleotide
atatctattatctggtcagttggcttatctaatctttccttaccgcac

SEQ ID NO: 26 - DNA, 34 bp, Artificial
  Synthetic Polynucleotide
cgcgaactgattggcacagacaatatatggaaat

SEQ ID NO: 27 - DNA, 32 bp, Artificial
  Synthetic Polynucleotide
attttccctcaaaagaaaaggctccaaaagga

SEQ ID NO: 28 - DNA, 30 bp, Artificial
  Synthetic Polynucleotide
cgtaatctgccaacggccacagttgaggat

SEQ ID NO: 29 - DNA, 40 bp, Artificial
  Synthetic Polynucleotide
cagcgtggtgctgcaggtcattggaaaccaaaagtaagag

SEQ ID NO: 30 - DNA, 40 bp, Artificial
  Synthetic Polynucleotide
gctatatgtgagtgaaaatttcttatagcccgagatagta

SEQ ID NO: 31 - DNA, 40 bp, Artificial
  Synthetic Polynucleotide
tttccagtaatgagtgagctaactgagccggaagcataaa

SEQ ID NO: 32 - DNA, 38 bp, Artificial
  Synthetic Polynucleotide
tttcccgttcaactttaatcattttatgcgattgtaaa

SEQ ID NO: 33 - DNA, 44 bp, Artificial
  Synthetic Polynucleotide
atagctggaaattggaggtttccctcagaacagtatatatacgc

SEQ ID NO: 34 - DNA, 48 bp, Artificial
  Synthetic Polynucleotide
agttttaagacgataatctggtcacaaccagcttacggctatgccggg

SEQ ID NO: 35 - DNA, 46 bp, Artificial
  Synthetic Polynucleotide
gcgcatcggcactcaatccgccgggcaacgggaacagcggttgcgg

SEQ ID NO: 36 - DNA, 39 bp, Artificial
  Synthetic Polynucleotide
ataggtcacgttggtgggagcaaagagcggaatcgtcat

SEQ ID NO: 37 - DNA, 32 bp, Artificial
  Synthetic Polynucleotide
gaggaaggaaatcaacgaaaccaaccgttgcc

SEQ ID NO: 38 - DNA, 36 bp, Artificial
  Synthetic Polynucleotide
aaattaaacgccaccctcaatcaatagtctttaatg

SEQ ID NO: 39 - DNA, 32 bp, Artificial
  Synthetic Polynucleotide
tacataaatcaattagttatcagcatcaatag

SEQ ID NO: 40 - DNA, 31 bp, Artificial
  Synthetic Polynucleotide
gggtgcctcgggaaacctaaacatagcgata

SEQ ID NO: 41 - DNA, 32 bp, Artificial
  Synthetic Polynucleotide
tcagaggggacgacgattttgccatagtaaaa

SEQ ID NO: 42 - DNA, 40 bp, Artificial
  Synthetic Polynucleotide
tgctgatctttaggagtagataatcagagggttttgaacc

SEQ ID NO: 43 - DNA, 48 bp, Artificial
  Synthetic Polynucleotide
tgacctttaattaattcatatggtcggcttagataactatatggaatt

SEQ ID NO: 44 - DNA, 30 bp, Artificial
  Synthetic Polynucleotide
gctcacaaaacgcggtccgtttaagggtaa

SEQ ID NO: 45 - DNA, 32 bp, Artificial
  Synthetic Polynucleotide
cggcctcaggaagcgctggcagcctccggtcc

SEQ ID NO: 46 - DNA, 31 bp, Artificial
  Synthetic Polynucleotide
ctagtcagaggcgaagagcccaacgctaacg

SEQ ID NO: 47 - DNA, 39 bp, Artificial
  Synthetic Polynucleotide
tcatatgctcatttggtgtaaagagacgttagagtgaga

SEQ ID NO: 48 - DNA, 48 bp, Artificial
  Synthetic Polynucleotide
ccgccagcaccctcatgaaacagcaaaaaaatcccgtaaaatttgtac

SEQ ID NO: 49 - DNA, 40 bp, Artificial
  Synthetic Polynucleotide
ggttggccgttccggcattccacatttcgccaagtacgct

SEQ ID NO: 50 - DNA, 32 bp, Artificial
  Synthetic Polynucleotide
cgtatcgcactccagcggataagtagctcaaa

SEQ ID NO: 51 - DNA, 29 bp, Artificial
  Synthetic Polynucleotide
gagggtaagagatccgtccaatactgaat

SEQ ID NO: 52 - DNA, 40 bp, Artificial
  Synthetic Polynucleotide
gaggatttagaagtatttaaatccaattgagctgagttaa

SEQ ID NO: 53 - DNA, 48 bp, Artificial
  Synthetic Polynucleotide
gtgccacgtttgcacgagcctaatttgccctgaacaagcacatcacct

SEQ ID NO: 54 - DNA, 48 bp, Artificial
  Synthetic Polynucleotide
acctttttaaccaagaaacatctcttaaaacgaaaagccagcgccaaa

SEQ ID NO: 55 - DNA, 40 bp, Artificial
  Synthetic Polynucleotide
atcgacatggatcaaacttaaattgagacgcatttgtaac

SEQ ID NO: 56 - DNA, 46 bp, Artificial
  Synthetic Polynucleotide
agttaaacgatgctgaaaagccgagaaccgcatgtaccgtaacgga

SEQ ID NO: 57 - DNA, 40 bp, Artificial
  Synthetic Polynucleotide
cgcttctgccaggcaagccgtcgagaaccgcctccctcag

SEQ ID NO: 58 - DNA, 31 bp, Artificial
  Synthetic Polynucleotide
tgcaaccgttctagctgatactttccggcac

SEQ ID NO: 59 - DNA, 30 bp, Artificial
  Synthetic Polynucleotide
tcaccatcaatatgatattcgggtcaggtt

SEQ ID NO: 60 - DNA, 40 bp, Artificial
  Synthetic Polynucleotide
ggttagcccgaacgttattttgcgtaataagattagagag

SEQ ID NO: 61 - DNA, 40 bp, Artificial
  Synthetic Polynucleotide
agaaataatagattttatattatttatccagcgcattaga

SEQ ID NO: 62 - DNA, 46 bp, Artificial
  Synthetic Polynucleotide
attcatttcaacatatcaaagacaccacggtctttccagtaacaaa

SEQ ID NO: 63 - DNA, 48 bp, Artificial
  Synthetic Polynucleotide
tggtgaagagacggtctgtagcatgacaacgtcaccaatggtacaacg

SEQ ID NO: 64 - DNA, 40 bp, Artificial
  Synthetic Polynucleotide
attcgccagcaactgtcgccaccccaccctcagagcccat

SEQ ID NO: 65 - DNA, 30 bp, Artificial
  Synthetic Polynucleotide
aaaaaagggtgagaataggattagcgggtg

SEQ ID NO: 66 - DNA, 32 bp, Artificial
  Synthetic Polynucleotide
ctgttgcgagaaaaataccagttacaaaataa

SEQ ID NO: 67 - DNA, 40 bp, Artificial
  Synthetic Polynucleotide
atcgcgcagaggctaaaacatgttgcagtcgatcaccgtc

SEQ ID NO: 68 - DNA, 44 bp, Artificial
  Synthetic Polynucleotide
gaggcgcggatagcctcataggatctaaagtttatttatcaaaa

SEQ ID NO: 69 - DNA, 45 bp, Artificial
  Synthetic Polynucleotide
aactttgatgagtttccaccgtaacagaataccggatattcacgg

SEQ ID NO: 70 - DNA, 48 bp, Artificial
  Synthetic Polynucleotide
gtagctgcttcagcagcaccaccggagggttgagcccggaataggtaa

SEQ ID NO: 71 - DNA, 50 bp, Artificial
  Synthetic Polynucleotide
ttttagaaccctcgcaaaattaagcaatagcaaggcaaagaattaatata

SEQ ID NO: 72 - DNA, 32 bp, Artificial
  Synthetic Polynucleotide
cagtaacacatcgggataaataaggcgccagt

SEQ ID NO: 73 - DNA, 32 bp, Artificial
  Synthetic Polynucleotide
caattgaataccaagtcttattacagcaaacg

SEQ ID NO: 74 - DNA, 32 bp, Artificial
  Synthetic Polynucleotide
tccatgtttatttgtatcatcgcctgataaat

SEQ ID NO: 75 - DNA, 45 bp, Artificial
  Synthetic Polynucleotide
ttttaaatgcaatgcctgagtaataagaggctgagtaactatttc

SEQ ID NO: 76 - DNA, 40 bp, Artificial
  Synthetic Polynucleotide
gcaattcatcattttagtaccataggacaatccaaataag

SEQ ID NO: 77 - DNA, 48 bp, Artificial
  Synthetic Polynucleotide
ttgctagaaatttaatggtttgaacagcagcgaaagacaggggagtta

SEQ ID NO: 78 - DNA, 36 bp, Artificial
  Synthetic Polynucleotide
aaactttttcaaataacttagcaaatatttccacag

SEQ ID NO: 79 - DNA, 40 bp, Artificial
  Synthetic Polynucleotide
cgggaacggatcagcttacgcaactttgccactcagacat

SEQ ID NO: 80 - DNA, 36 bp, Artificial
  Synthetic Polynucleotide
gagattttagttaatgcaacggaattattagcaaaa

SEQ ID NO: 81 - DNA, 40 bp, Artificial
  Synthetic Polynucleotide
cttcatcatgacaagacaagtttgcctttcattagcaagg

SEQ ID NO: 82 - DNA, 48 bp, Artificial
  Synthetic Polynucleotide
caatgtgctgcaaggcgatttcagaggtggagtgccatctctcaccgg

SEQ ID NO: 83 - DNA, 46 bp, Artificial
  Synthetic Polynucleotide
acatttcgattcccaattctgcggtacggtgtctggaaattctgta

SEQ ID NO: 84 - DNA, 24 bp, Artificial
  Synthetic Polynucleotide
aacatccaaggtgttagtctctga

SEQ ID NO: 85 - DNA, 48 bp, Artificial
  Synthetic Polynucleotide
aataacagaggcatttaataagagaaaaacagtaatcctgattgtcaa

SEQ ID NO: 86 - DNA, 47 bp, Artificial
  Synthetic Polynucleotide
tcgagttacgtcaaaaaggaaaccgaggaaacgcaataaggaaccgg

SEQ ID NO: 87 - DNA, 37 bp, Artificial
  Synthetic Polynucleotide
tcaccctataccgacaagactctaccagatgaatata

SEQ ID NO: 88 - DNA, 32 bp, Artificial
  Synthetic Polynucleotide
ccagtgccaagcttaaccatagccggtcacca

SEQ ID NO: 89 - DNA, 32 bp, Artificial
  Synthetic Polynucleotide
gatgcatcaattctactaaagccaattcacaa

SEQ ID NO: 90 - DNA, 48 bp, Artificial
  Synthetic Polynucleotide
aatcataattacaacaaacgcctagccaacgccacacgacgctcaatc

SEQ ID NO: 91 - DNA, 48 bp, Artificial
  Synthetic Polynucleotide
aaggccgctgccgcatgcccagttatacaaatggttttgaagcgttgc

SEQ ID NO: 92 - DNA, 45 bp, Artificial
  Synthetic Polynucleotide
aggctttgactttttcatgtaacgcctggccctgagagagttgca

SEQ ID NO: 93 - DNA, 40 bp, Artificial
  Synthetic Polynucleotide
tttcccagtcacgacgttgtaaaagcattttccccttatt

SEQ ID NO: 94 - DNA, 40 bp, Artificial
  Synthetic Polynucleotide
aaccagacctctttaacgcgtcaatcattaacattttaca

SEQ ID NO: 95 - DNA, 37 bp, Artificial
  Synthetic Polynucleotide
ctgtttagtatcatattttgcgtaacggaaaactggc

SEQ ID NO: 96 - DNA, 32 bp, Artificial
  Synthetic Polynucleotide
cgcctaaagaggatgattagagcccattaaag

SEQ ID NO: 97 - DNA, 48 bp, Artificial
  Synthetic Polynucleotide
acgttaattttaggaatgtcactgagccagcggtgccggtgtggtgcc

SEQ ID NO: 98 - DNA, 40 bp, Artificial
  Synthetic Polynucleotide
acaacattgtttcatttgacaggattattctgaaagccac

SEQ ID NO: 99 - DNA, 47 bp, Artificial
  Synthetic Polynucleotide
gctcaacatgttttaaatgcaaacggaaatggccttgatgaatggaa

SEQ ID NO: 100 - DNA, 39 bp, Artificial
  Synthetic Polynucleotide
ccagtcaggagcttgccctgacgagaaggcagaaagaac

SEQ ID NO: 101 - DNA, 39 bp, Artificial
  Synthetic Polynucleotide
gattattgctgaatataatgacaggtagaaagccaaaag

SEQ ID NO: 102 - DNA, 24 bp, Artificial
  Synthetic Polynucleotide
taatataattacaatatgtagcat

SEQ ID NO: 103 - DNA, 40 bp, Artificial
  Synthetic Polynucleotide
agcgaacccagatataaaacgctcttttgaatggccagaa

SEQ ID NO: 104 - DNA, 46 bp, Artificial
  Synthetic Polynucleotide
gccgacaatgaatacgtaatgccactacgaattgaaaatctccaaa

SEQ ID NO: 105 - DNA, 40 bp, Artificial
  Synthetic Polynucleotide
accagaacgagtattagcagcgtgcctgttcttcgttttc

SEQ ID NO: 106 - DNA, 29 bp, Artificial
  Synthetic Polynucleotide
gaatggcttagagcttgcggctaaaggtt

SEQ ID NO: 107 - DNA, 48 bp, Artificial
  Synthetic Polynucleotide
attagagggattagctccttttgacaaatgctttaaagaattaatggg

SEQ ID NO: 108 - DNA, 32 bp, Artificial
  Synthetic Polynucleotide
aaaaacagcttgataccgatacttagcgggtt

SEQ ID NO: 109 - DNA, 31 bp, Artificial
  Synthetic Polynucleotide
ttttcacgggcaccaaagtggcgaaaatcct

SEQ ID NO: 110 - DNA, 45 bp, Artificial
  Synthetic Polynucleotide
ttgggcttccgtgagcctcctagcaccgtcggccccctagaactg

SEQ ID NO: 111 - DNA, 40 bp, Artificial
  Synthetic Polynucleotide
ctcttaccgtgaagttgtactcagttaccagagcacatcc

SEQ ID NO: 112 - DNA, 48 bp, Artificial
  Synthetic Polynucleotide
caacactaaatgcagatacataacgattcatcgccagcatccaagggt

SEQ ID NO: 113 - DNA, 47 bp, Artificial
  Synthetic Polynucleotide
gcggattaccagccgggtcactgttgagtaagagcgccctaagagag

SEQ ID NO: 114 - DNA, 46 bp, Artificial
  Synthetic Polynucleotide
aatgttgattaagcaagcaaattcccgactattttgaccagtaata

SEQ ID NO: 115 - DNA, 45 bp, Artificial
  Synthetic Polynucleotide
cacccgtgtaaccttgcttctcctaaaacataataccgtcctgaa

SEQ ID NO: 116 - DNA, 46 bp, Artificial
  Synthetic Polynucleotide
gccttagaaaggaacggggagaggcggtcccttataaattagaatc

SEQ ID NO: 117 - DNA, 30 bp, Artificial
  Synthetic Polynucleotide
tcattgaatcccccttaagaggtcattttt

SEQ ID NO: 118 - DNA, 32 bp, Artificial
  Synthetic Polynucleotide
gagagctacaattttaaacgaaccaccagcag

SEQ ID NO: 119 - DNA, 40 bp, Artificial
  Synthetic Polynucleotide
tttcagcggtaaatgaattttctggagccaccagttgggc

SEQ ID NO: 120 - DNA, 40 bp, Artificial
  Synthetic Polynucleotide
aaacaactgtttaatttgcgctcagtaccgagctcgaatt

SEQ ID NO: 121 - DNA, 48 bp, Artificial
  Synthetic Polynucleotide
cagaaaaccaagagaagtaatcgtaaattttggctatacttaacgggg

SEQ ID NO: 122 - DNA, 32 bp, Artificial
  Synthetic Polynucleotide
agcgaataagtttattttgtcacattgctttc

SEQ ID NO: 123 - DNA, 40 bp, Artificial
  Synthetic Polynucleotide
gaccataaataagtttagcatgtcgaccctgtaatacttt

SEQ ID NO: 124 - DNA, 29 bp, Artificial
  Synthetic Polynucleotide
caccctccacaggcttaccagtcccggaa

SEQ ID NO: 125 - DNA, 46 bp, Artificial
  Synthetic Polynucleotide
ttgctcagctggatagtacaaaggattgcctgagagtcttagatgg

SEQ ID NO: 126 - DNA, 40 bp, Artificial
  Synthetic Polynucleotide
tactggtaatcaaaaacccgaacgtcgataaaaacaggaa

SEQ ID NO: 127 - DNA, 46 bp, Artificial
  Synthetic Polynucleotide
gacaagcctctgttatgttggcacggaaaaatcggtctgagagact

SEQ ID NO: 128 - DNA, 40 bp, Artificial
  Synthetic Polynucleotide
ttagccagggatagcaacaacgccaatcataacgacctgc

SEQ ID NO: 129 - DNA, 48 bp, Artificial
  Synthetic Polynucleotide
aggaaccccaccctcatatgggatcaacataccacattaattgtgtgt

SEQ ID NO: 130 - DNA, 40 bp, Artificial
  Synthetic Polynucleotide
ctcagaactgggaaggcgggcctcttcgctatggcgaaag

SEQ ID NO: 131 - DNA, 38 bp, Artificial
  Synthetic Polynucleotide
aaacgattcgtgtgagaaacaataacggattcgcctga

SEQ ID NO: 132 - DNA, 32 bp, Artificial
  Synthetic Polynucleotide
gatagcaggtcaccagtacaaactagcccaat

SEQ ID NO: 133 - DNA, 39 bp, Artificial
  Synthetic Polynucleotide
gaaagtattgtcggtggcgatgtaggtaaagattcaaat

SEQ ID NO: 134 - DNA, 32 bp, Artificial
  Synthetic Polynucleotide
atttaccgcgtcatacatgtgcccgtataaac

SEQ ID NO: 135 - DNA, 40 bp, Artificial
  Synthetic Polynucleotide
gtgaattattgagggagggaaggtcggtccaatcgcaaga

SEQ ID NO: 136 - DNA, 48 bp, Artificial
  Synthetic Polynucleotide
ccggaggactaataccaagcgcgaaacaatctagagtaaaaaaccatc

SEQ ID NO: 137 - DNA, 40 bp, Artificial
  Synthetic Polynucleotide
cagaaccagttgggtaacgcctataacagttgcaaatggt

SEQ ID NO: 138 - DNA, 47 bp, Artificial
  Synthetic Polynucleotide
ggaacctaggttgaggcaggtcagacgattgcaactaaaaacgagta

SEQ ID NO: 139 - DNA, 48 bp, Artificial
  Synthetic Polynucleotide
agccctgctgcccgcagtttgaccggggcgcgagctgaaaataaatca

SEQ ID NO: 140 - DNA, 38 bp, Artificial
  Synthetic Polynucleotide
tcaccagtcacaggaagtttccatttgccccagcagag

SEQ ID NO: 141 - DNA, 46 bp, Artificial
  Synthetic Polynucleotide
agcgcgttttcatcgcgattacccaaatcaacgtaacattcagtga

SEQ ID NO: 142 - DNA, 30 bp, Artificial
  Synthetic Polynucleotide
aaagggaaccgtctatcattataatcagtg

SEQ ID NO: 143 - DNA, 32 bp, Artificial
  Synthetic Polynucleotide
tattaaagaaccggtcgcaaggtgtattcggt

SEQ ID NO: 144 - DNA, 31 bp, Artificial
  Synthetic Polynucleotide
tcttagcctcctgttgctcgtcataaacatc

SEQ ID NO: 145 - DNA, 40 bp, Artificial
  Synthetic Polynucleotide
ttacctgccgcgcctgtgctgttctggtgactctaacgga

SEQ ID NO: 146 - DNA, 39 bp, Artificial
  Synthetic Polynucleotide
cttgagtcgtgccagctgcattaatgaacggctgcccgc

SEQ ID NO: 147 - DNA, 37 bp, Artificial
  Synthetic Polynucleotide
agaggtgtattaacacctacatttaatgcctgcaaca

SEQ ID NO: 148 - DNA, 32 bp, Artificial
  Synthetic Polynucleotide
ttcatttgtttaatggaaacagaagataaaac

SEQ ID NO: 149 - DNA, 32 bp, Artificial
  Synthetic Polynucleotide
agaagatgatgaaacaaaacaaaattaacaat

SEQ ID NO: 150 - DNA, 40 bp, Artificial
  Synthetic Polynucleotide
agaagcctttattagctaaatcggaacattataatcatat

SEQ ID NO: 151 - DNA, 30 bp, Artificial
  Synthetic Polynucleotide
aaacaggacagatgagaccaggcgcatcca

SEQ ID NO: 152 - DNA, 38 bp, Artificial
  Synthetic Polynucleotide
ggggataacctgtttagctatattttcatttattagat

SEQ ID NO: 153 - DNA, 32 bp, Artificial
  Synthetic Polynucleotide
cgagggtattcatcttctgacctaacgcgaga

SEQ ID NO: 154 - DNA, 32 bp, Artificial
  Synthetic Polynucleotide
tctgctcaaagctttgacccccagcgattcag

SEQ ID NO: 155 - DNA, 48 bp, Artificial
  Synthetic Polynucleotide
ataagcgtgttttcacggtcataccgggattgcccttcacaacactca

SEQ ID NO: 156 - DNA, 40 bp, Artificial
  Synthetic Polynucleotide
tcttacgtttttattttcatcctgaataacctcaaatatc

SEQ ID NO: 157 - DNA, 30 bp, Artificial
  Synthetic Polynucleotide
attaattgtatcggtattaagacgctgatg

SEQ ID NO: 158 - DNA, 40 bp, Artificial
  Synthetic Polynucleotide
gagggggtgtatcacctaccagaccggaacgtgccgggtc

SEQ ID NO: 159 - DNA, 32 bp, Artificial
  Synthetic Polynucleotide
aaatttgcaaaagaagcagaggtcctatctat

SEQ ID NO: 160 - DNA, 32 bp, Artificial
  Synthetic Polynucleotide
tcatcgagaacaaagtacagcaaatgaaaaat

SEQ ID NO: 161 - DNA, 30 bp, Artificial
  Synthetic Polynucleotide
aaatgtcgtctttccccgaagagtcaatag

SEQ ID NO: 162 - DNA, 32 bp, Artificial
  Synthetic Polynucleotide
tgtttagataccaggccagaattaatgccgga

SEQ ID NO: 163 - DNA, 48 bp, Artificial
  Synthetic Polynucleotide
aactgaacaatggaagtaccatatcaaaattactgagagccagcattt

SEQ ID NO: 164 - DNA, 48 bp, Artificial
  Synthetic Polynucleotide
accagagccgccatgtggcctttagtgggaaagtgccatgtttcgtct

SEQ ID NO: 165 - DNA, 32 bp, Artificial
  Synthetic Polynucleotide
atgattttttgtttaaaataagaataaactcg

SEQ ID NO: 166 - DNA, 48 bp, Artificial
  Synthetic Polynucleotide
accaaaagtacccgacttgagccacaaccatcaaccgatagactccaa

SEQ ID NO: 167 - DNA, 31 bp, Artificial
  Synthetic Polynucleotide
agctagcgatcaggttccgaggctggctgac

SEQ ID NO: 168 - DNA, 48 bp, Artificial
  Synthetic Polynucleotide
ttaccagaatgaaaatagcagcctaataacataatataaaagatgatg

SEQ ID NO: 169 - DNA, 40 bp, Artificial
  Synthetic Polynucleotide
gagccgccagttgagaaaaacgaactgtggtgctgcggcc

SEQ ID NO: 170 - DNA, 32 bp, Artificial
  Synthetic Polynucleotide
aactgacctttgtgagagatagactttctccg

SEQ ID NO: 171 - DNA, 32 bp, Artificial
  Synthetic Polynucleotide
tgtgtacaacggtgtcgaaatccggggaaccg

SEQ ID NO: 172 - DNA, 32 bp, Artificial
  Synthetic Polynucleotide
gccgaattcgggacaagaattggattatactt

SEQ ID NO: 173 - DNA, 30 bp, Artificial
  Synthetic Polynucleotide
acaacataaaggtggcaattacctgagaac

SEQ ID NO: 174 - DNA, 32 bp, Artificial
  Synthetic Polynucleotide
ccttgagtaacaggcttaatcaacgcaaggat

SEQ ID NO: 175 - DNA, 30 bp, Artificial
  Synthetic Polynucleotide
tagaaaatacatgcccaggtttaacgtaaa

SEQ ID NO: 176 - DNA, 32 bp, Artificial
  Synthetic Polynucleotide
acaaagggcgacattcatgctgatgcaaaaac

SEQ ID NO: 177 - DNA, 30 bp, Artificial
  Synthetic Polynucleotide
aatcaaaatcaccacaagaatcggcgaaac

SEQ ID NO: 178 - DNA, 47 bp, Artificial
  Synthetic Polynucleotide
agtactcctcaagagaagccaccagccggataggccggagacaggcc

SEQ ID NO: 179 - DNA, 30 bp, Artificial; identical to SEQ ID NO: 142
  Synthetic Polynucleotide

SEQ ID NO: 180 - DNA, 32 bp, Artificial; identical to SEQ ID NO: 143
  Synthetic Polynucleotide

SEQ ID NO: 181 - DNA, 31 bp, Artificial; identical to SEQ ID NO: 144
  Synthetic Polynucleotide

SEQ ID NO: 182 - DNA, 40 bp, Artificial; identical to SEQ ID NO: 145
  Synthetic Polynucleotide

SEQ ID NO: 183 - DNA, 39 bp, Artificial; identical to SEQ ID NO: 146
  Synthetic Polynucleotide

SEQ ID NO: 184 - DNA, 37 bp, Artificial; identical to SEQ ID NO: 147
  Synthetic Polynucleotide

SEQ ID NO: 185 - DNA, 32 bp, Artificial; identical to SEQ ID NO: 148
  Synthetic Polynucleotide

SEQ ID NO: 186 - DNA, 32 bp, Artificial; identical to SEQ ID NO: 149
  Synthetic Polynucleotide

SEQ ID NO: 187 - DNA, 40 bp, Artificial; identical to SEQ ID NO: 150
  Synthetic Polynucleotide

SEQ ID NO: 188 - DNA, 30 bp, Artificial; identical to SEQ ID NO: 151
  Synthetic Polynucleotide

SEQ ID NO: 189 - DNA, 38 bp, Artificial; identical to SEQ ID NO: 152
  Synthetic Polynucleotide

SEQ ID NO: 190 - DNA, 32 bp, Artificial; identical to SEQ ID NO: 153
  Synthetic Polynucleotide

SEQ ID NO: 191 - DNA, 32 bp, Artificial; identical to SEQ ID NO: 154
  Synthetic Polynucleotide

SEQ ID NO: 192 - DNA, 48 bp, Artificial; identical to SEQ ID NO: 155
  Synthetic Polynucleotide

SEQ ID NO: 193 - DNA, 40 bp, Artificial; identical to SEQ ID NO: 156
  Synthetic Polynucleotide

SEQ ID NO: 194 - DNA, 30 bp, Artificial; identical to SEQ ID NO: 157
  Synthetic Polynucleotide

SEQ ID NO: 195 - DNA, 40 bp, Artificial; identical to SEQ ID NO: 158
  Synthetic Polynucleotide

SEQ ID NO: 196 - DNA, 32 bp, Artificial; identical to SEQ ID NO: 159
  Synthetic Polynucleotide

SEQ ID NO: 197 - DNA, 32 bp, Artificial; identical to SEQ ID NO: 160
  Synthetic Polynucleotide

SEQ ID NO: 198 - DNA, 30 bp, Artificial; identical to SEQ ID NO: 161
  Synthetic Polynucleotide

SEQ ID NO: 199 - DNA, 32 bp, Artificial; identical to SEQ ID NO: 162
  Synthetic Polynucleotide

SEQ ID NO: 200 - DNA, 48 bp, Artificial; identical to SEQ ID NO: 163
  Synthetic Polynucleotide

SEQ ID NO: 201 - DNA, 48 bp, Artificial; identical to SEQ ID NO: 164
  Synthetic Polynucleotide

SEQ ID NO: 202 - DNA, 32 bp, Artificial; identical to SEQ ID NO: 165
  Synthetic Polynucleotide

SEQ ID NO: 203 - DNA, 48 bp, Artificial; identical to SEQ ID NO: 166
  Synthetic Polynucleotide

SEQ ID NO: 204 - DNA, 31 bp, Artificial; identical to SEQ ID NO: 167
  Synthetic Polynucleotide

SEQ ID NO: 205 - DNA, 48 bp, Artificial; identical to SEQ ID NO: 168
  Synthetic Polynucleotide

SEQ ID NO: 206 - DNA, 40 bp, Artificial; identical to SEQ ID NO: 169
  Synthetic Polynucleotide

SEQ ID NO: 207 - DNA, 42 bp, Artificial
  Synthetic Polynucleotide
ttgattaaatcagctccaataggaacgaattaaccgtcttct

SEQ ID NO: 208 - DNA, 38 bp, Artificial
  Synthetic Polynucleotide
tgagtagaagatagatcgagcatgtaagttgaatataa

SEQ ID NO: 209 - DNA, 29 bp, Artificial
  Synthetic Polynucleotide
ccgtaaattgtaaacgttaaactcaaact

SEQ ID NO: 210 - DNA, 45 bp, Artificial
  Synthetic Polynucleotide
gcaaatatgcaaagcgttttgttataaatttttgttagtaataac

SEQ ID NO: 211 - DNA, 42 bp, Artificial
  Synthetic Polynucleotide
gattgtaatcagaaaagctcaggtcttattatagtcacagtt

SEQ ID NO: 212 - DNA, 39 bp, Artificial
  Synthetic Polynucleotide
gtaccccggttgatacaaacaccaaattgtaattcgaca

SEQ ID NO: 213 - DNA, 45 bp, Artificial
  Synthetic Polynucleotide
actcgtatagacttgattagagccgtcaacactaacaaaaccaag

SEQ ID NO: 214 - DNA, 41 bp, Artificial
  Synthetic Polynucleotide
cattatcattaattcaagaatgctaatatcagagaggagtg

SEQ ID NO: 215 - DNA, 44 bp, Artificial
  Synthetic Polynucleotide
agaaaccatgattatcgtaccgacaaaaggtaaagtgtagcatt

SEQ ID NO: 216 - DNA, 41 bp, Artificial
  Synthetic Polynucleotide
tacagttatcatcatattccccagaagagctatcgcaagaa

SEQ ID NO: 217 - DNA, 43 bp, Artificial
  Synthetic Polynucleotide
tgtccagaagccctttttaatcctcattaatagtatcaaagcg

SEQ ID NO: 218 - DNA, 41 bp, Artificial
  Synthetic Polynucleotide
gcgcctgtttatcaacagaggagtctgtccatcacgcacca

SEQ ID NO: 219 - DNA, 42 bp, Artificial
  Synthetic Polynucleotide
tcctaatttatgcatcaaaaaaagcccgaaagacaagaaaaa

SEQ ID NO: 220 - DNA, 46 bp, Artificial
  Synthetic Polynucleotide
tatcattccaagaacctgacttaccgggtattactaataaggaatt

SEQ ID NO: 221 - DNA, 42 bp, Artificial
  Synthetic Polynucleotide
tgatacaggtaagttccaatagcaatgagcggaattgagtaa

SEQ ID NO: 222 - DNA, 42 bp, Artificial
  Synthetic Polynucleotide
acaatgaaataacccattaaaagtaagcctcagagcatttga

SEQ ID NO: 223 - DNA, 41 bp, Artificial
  Synthetic Polynucleotide
ttacaccgacgacgacatgttcagctaatgcagaacaattc

SEQ ID NO: 224 - DNA, 41 bp, Artificial
  Synthetic Polynucleotide
agatagccattatagataagtcctgaactagaaaagtaagc

SEQ ID NO: 225 - DNA, 32 bp, Artificial
  Synthetic Polynucleotide
acaaataatcaaatatttcgagcttcaaaaat

SEQ ID NO: 226 - DNA, 53 bp, Artificial
  Synthetic Polynucleotide
aactgacctttgtgagagatagactttctccgcggttgtactgtgaccgattc

SEQ ID NO: 227 - DNA, 53 bp, Artificial
  Synthetic Polynucleotide
tgtgtacaacggtgtcgaaatccggggaaccgcggttgtactgtgaccgattc

SEQ ID NO: 228 - DNA, 53 bp, Artificial
  Synthetic Polynucleotide
gccgaattcgggacaagaattggattatacttcggttgtactgtgaccgattc

SEQ ID NO: 229 - DNA, 51 bp, Artificial
  Synthetic Polynucleotide
acaacataaaggtggcaattacctgagaaccggttgtactgtgaccgattc

SEQ ID NO: 230 - DNA, 53 bp, Artificial
  Synthetic Polynucleotide
ccttgagtaacaggcttaatcaacgcaaggatcggttgtactgtgaccgattc

SEQ ID NO: 231 - DNA, 51 bp, Artificial
  Synthetic Polynucleotide
tagaaaatacatgcccaggtttaacgtaaacggttgtactgtgaccgattc

SEQ ID NO: 232 - DNA, 53 bp, Artificial
  Synthetic Polynucleotide
acaaagggcgacattcatgctgatgcaaaaaccggttgtactgtgaccgattc

SEQ ID NO: 233 - DNA, 51 bp, Artificial
  Synthetic Polynucleotide
aatcaaaatcaccacaagaatcggcgaaaccggttgtactgtgaccgattc

SEQ ID NO: 234 - DNA, 68 bp, Artificial
  Synthetic Polynucleotide
agtactcctcaagagaagccaccagccggataggccggagacaggcccggttgtactgtgaccgattc

SEQ ID NO: 235 - DNA, 44 bp, Artificial
  Synthetic Polynucleotide
taaatgaattttctgtatgggattaatttcttttgatctacata

SEQ ID NO: 236 - DNA, 43 bp, Artificial
  Synthetic Polynucleotide
tctaaagttttgtcgtctttccagccgacaattgatctacata

SEQ ID NO: 237 - DNA, 44 bp, Artificial
  Synthetic Polynucleotide
tccacagacagccctcatagttagcgtaacgattgatctacata

SEQ ID NO: 238 - DNA, 44 bp, Artificial
  Synthetic Polynucleotide
tcaccagtacaaactacaacgcctagtaccagttgatctacata

SEQ ID NO: 239 - DNA, 43 bp, Artificial
  Synthetic Polynucleotide
aggaacccatgtaccgtaacacttgatataattgatctacata

SEQ ID NO: 240 - DNA, 42 bp, Artificial
  Synthetic Polynucleotide
aggctccagaggctttgaggacacgggtaattgatctacata

SEQ ID NO: 241 - DNA, 44 bp, Artificial
  Synthetic Polynucleotide
aaacagctttttgcgggatcgtcaacactaaattgatctacata

SEQ ID NO: 242 - DNA, 42 bp, Artificial
  Synthetic Polynucleotide
gtatagcaaacagttaatgcccaatcctcattgatctacata

SEQ ID NO: 243 - DNA, 42 bp, Artificial
  Synthetic Polynucleotide
cagcgaaacttgctttcgaggtgttgctaattgatctacata

SEQ ID NO: 244 - DNA, 44 bp, Artificial
  Synthetic Polynucleotide
aaggccgctgataccgatagttgcgacgttagttgatctacata

SEQ ID NO: 245 - DNA, 44 bp, Artificial
  Synthetic Polynucleotide
atattcggaaccatcgcccacgcagagaaggattgatctacata

SEQ ID NO: 246 - DNA, 42 bp, Artificial
  Synthetic Polynucleotide
tattaagaagcggggttttgctcgtagcatttgatctacata

SEQ ID NO: 247 - DNA, 44 bp, Artificial
  Synthetic Polynucleotide
tttcggaagtgccgtcgagagggtgagtttcgttgatctacata

SEQ ID NO: 248 - DNA, 42 bp, Artificial
  Synthetic Polynucleotide
aatacgtttgaaagaggacagactgaccttttgatctacata

SEQ ID NO: 249 - DNA, 44 bp, Artificial
  Synthetic Polynucleotide
acactcatccatgttacttagccgaaagctgcttgatctacata

SEQ ID NO: 250 - DNA, 44 bp, Artificial
  Synthetic Polynucleotide
ttgacaggccaccaccagagccgcgatttgtattgatctacata

SEQ ID NO: 251 - DNA, 42 bp, Artificial
  Synthetic Polynucleotide
ttaaagccagagccgccaccctcgacagaattgatctacata

SEQ ID NO: 252 - DNA, 44 bp, Artificial
  Synthetic Polynucleotide
tcatcgccaacaaagtacaacggacgccagcattgatctacata

SEQ ID NO: 253 - DNA, 42 bp, Artificial
  Synthetic Polynucleotide
catcaagtaaaacgaactaacgagttgagattgatctacata

SEQ ID NO: 254 - DNA, 44 bp, Artificial
  Synthetic Polynucleotide
tcattcagatgcgattttaagaacaggcatagttgatctacata

SEQ ID NO: 255 - DNA, 42 bp, Artificial
  Synthetic Polynucleotide
tcaagtttcattaaaggtgaatataaaagattgatctacata

SEQ ID NO: 256 - DNA, 44 bp, Artificial
  Synthetic Polynucleotide
tacgttaaagtaatcttgacaagaaccgaactttgatctacata

SEQ ID NO: 257 - DNA, 42 bp, Artificial
  Synthetic Polynucleotide
ttataccaccaaatcaacgtaacgaacgagttgatctacata

SEQ ID NO: 258 - DNA, 44 bp, Artificial
  Synthetic Polynucleotide
attacctttgaataaggcttgcccaaatccgcttgatctacata

SEQ ID NO: 259 - DNA, 44 bp, Artificial
  Synthetic Polynucleotide
gatggtttgaacgagtagtaaatttaccattattgatctacata

SEQ ID NO: 260 - DNA, 42 bp, Artificial
  Synthetic Polynucleotide
cagcaaaaggaaacgtcaccaatgagccgcttgatctacata

SEQ ID NO: 261 - DNA, 44 bp, Artificial
  Synthetic Polynucleotide
tcaccgacgcaccgtaatcagtagcagaaccgttgatctacata

SEQ ID NO: 262 - DNA, 44 bp, Artificial
  Synthetic Polynucleotide
gaaattattgcctttagcgtcagaccggaaccttgatctacata

SEQ ID NO: 263 - DNA, 42 bp, Artificial
  Synthetic Polynucleotide
accgattgtcggcattttcggtcataatcattgatctacata

SEQ ID NO: 264 - DNA, 42 bp, Artificial
  Synthetic Polynucleotide
tttaggacaaatgctttaaacaatcaggtcttgatctacata

SEQ ID NO: 265 - DNA, 44 bp, Artificial
  Synthetic Polynucleotide
taagagcaaatgtttagactggataggaagccttgatctacata

SEQ ID NO: 266 - DNA, 44 bp, Artificial
  Synthetic Polynucleotide
ttattacgaagaactggcatgattgcgagaggttgatctacata

SEQ ID NO: 267 - DNA, 42 bp, Artificial
  Synthetic Polynucleotide
aacgcaaagatagccgaacaaaccctgaacttgatctacata

SEQ ID NO: 268 - DNA, 44 bp, Artificial
  Synthetic Polynucleotide
cttttgcagataaaaaccaaaataaagactccttgatctacata

SEQ ID NO: 269 - DNA, 42 bp, Artificial
  Synthetic Polynucleotide
tttaccccaacatgttttaaatttccatatttgatctacata

SEQ ID NO: 270 - DNA, 44 bp, Artificial
  Synthetic Polynucleotide
cggattgcagagcttaattgctgaaacgagtattgatctacata

SEQ ID NO: 271 - DNA, 44 bp, Artificial
  Synthetic Polynucleotide
cgaaagactttgataagaggtcatatttcgcattgatctacata

SEQ ID NO: 272 - DNA, 42 bp, Artificial
  Synthetic Polynucleotide
gcttcaatcaggattagagagttattttcattgatctacata

SEQ ID NO: 273 - DNA, 44 bp, Artificial
  Synthetic Polynucleotide
ttagacggccaaataagaaacgatagaaggctttgatctacata

SEQ ID NO: 274 - DNA, 42 bp, Artificial
  Synthetic Polynucleotide
aaagtcacaaaataaacagccagcgttttattgatctacata

SEQ ID NO: 275 - DNA, 44 bp, Artificial
  Synthetic Polynucleotide
gagagatagagcgtctttccagaggttttgaattgatctacata

SEQ ID NO: 276 - DNA, 44 bp, Artificial
  Synthetic Polynucleotide
ctgtagcttgactattatagtcagttcattgattgatctacata

SEQ ID NO: 277 - DNA, 42 bp, Artificial
  Synthetic Polynucleotide
gatggcttatcaaaaagattaagagcgtccttgatctacata

SEQ ID NO: 278 - DNA, 44 bp, Artificial
  Synthetic Polynucleotide
ttgctcctttcaaatatcgcgtttgagggggtttgatctacata

SEQ ID NO: 279 - DNA, 44 bp, Artificial
  Synthetic Polynucleotide
ccaacaggagcgaaccagaccggagcctttacttgatctacata

SEQ ID NO: 280 - DNA, 42 bp, Artificial
  Synthetic Polynucleotide
ttaacgtctaacataaaaacaggtaacggattgatctacata

SEQ ID NO: 281 - DNA, 44 bp, Artificial
  Synthetic Polynucleotide
atcccaatgagaattaactgaacagttaccagttgatctacata

SEQ ID NO: 282 - DNA, 44 bp, Artificial
  Synthetic Polynucleotide
gccagttagagggtaattgagcgctttaagaattgatctacata

SEQ ID NO: 283 - DNA, 42 bp, Artificial
  Synthetic Polynucleotide
acgctaacacccacaagaattgaaaatagcttgatctacata

SEQ ID NO: 284 - DNA, 44 bp, Artificial
  Synthetic Polynucleotide
ttctactacgcgagctgaaaaggttaccgcgcttgatctacata

SEQ ID NO: 285 - DNA, 42 bp, Artificial
  Synthetic Polynucleotide
aacgcaaaatcgatgaacggtaccggttgattgatctacata

SEQ ID NO: 286 - DNA, 44 bp, Artificial
  Synthetic Polynucleotide
tatattttgtcattgcctgagagtggaagattttgatctacata

SEQ ID NO: 287 - DNA, 44 bp, Artificial
  Synthetic Polynucleotide
taggtaaactatttttgagagatcaaacgttattgatctacata

SEQ ID NO: 288 - DNA, 42 bp, Artificial
  Synthetic Polynucleotide
gagacagctagctgataaattaatttttgtttgatctacata

SEQ ID NO: 289 - DNA, 44 bp, Artificial
  Synthetic Polynucleotide
gtaaagtaatcgccatatttaacaaaacttttttgatctacata

SEQ ID NO: 290 - DNA, 42 bp, Artificial
  Synthetic Polynucleotide
acaacatgccaacgctcaacagtcttctgattgatctacata

SEQ ID NO: 291 - DNA, 44 bp, Artificial
  Synthetic Polynucleotide
gtttatcaatatgcgttatacaaaccgaccgtttgatctacata

SEQ ID NO: 292 - DNA, 42 bp, Artificial
  Synthetic Polynucleotide
ttagtatcacaatagataagtccacgagcattgatctacata

SEQ ID NO: 293 - DNA, 42 bp, Artificial
  Synthetic Polynucleotide
taatcagcggattgaccgtaatcgtaaccgttgatctacata

SEQ ID NO: 294 - DNA, 44 bp, Artificial
  Synthetic Polynucleotide
atattttggctttcatcaacattatccagccattgatctacata

SEQ ID NO: 295 - DNA, 44 bp, Artificial
  Synthetic Polynucleotide
atcgcaagtatgtaaatgctgatgataggaacttgatctacata

SEQ ID NO: 296 - DNA, 42 bp, Artificial
  Synthetic Polynucleotide
cctaaatcaaaatcataggtctaaacagtattgatctacata

SEQ ID NO: 297 - DNA, 44 bp, Artificial
  Synthetic Polynucleotide
gccatcaagctcattttttaaccacaaatccattgatctacata

SEQ ID NO: 298 - DNA, 42 bp, Artificial
  Synthetic Polynucleotide
tgcatctttcccagtcacgacggcctgcagttgatctacata

SEQ ID NO: 299 - DNA, 44 bp, Artificial
  Synthetic Polynucleotide
gctttccgattacgccagctggcggctgtttcttgatctacata

SEQ ID NO: 300 - DNA, 42 bp, Artificial
  Synthetic Polynucleotide
cataaatctttgaataccaagtgttagaacttgatctacata

SEQ ID NO: 301 - DNA, 44 bp, Artificial
  Synthetic Polynucleotide
ccagggttgccagtttgaggggacccgtgggattgatctacata

SEQ ID NO: 302 - DNA, 42 bp, Artificial
  Synthetic Polynucleotide
gatgtgcttcaggaagatcgcacaatgtgattgatctacata

SEQ ID NO: 303 - DNA, 44 bp, Artificial
  Synthetic Polynucleotide
tcttcgctgcaccgcttctggtgcggccttccttgatctacata

SEQ ID NO: 304 - DNA, 44 bp, Artificial
  Synthetic Polynucleotide
caactgttgcgccattcgccattcaaacatcattgatctacata

SEQ ID NO: 305 - DNA, 42 bp, Artificial
  Synthetic Polynucleotide
ctgagcaaaaattaattacattttgggttattgatctacata

SEQ ID NO: 306 - DNA, 44 bp, Artificial
  Synthetic Polynucleotide
cgcgcagattaccttttttaatgggagagactttgatctacata

SEQ ID NO: 307 - DNA, 44 bp, Artificial
  Synthetic Polynucleotide
cctgattgcaatatatgtgagtgatcaatagtttgatctacata

SEQ ID NO: 308 - DNA, 42 bp, Artificial
  Synthetic Polynucleotide
cttttacaaaatcgtcgctattagcgatagttgatctacata

SEQ ID NO: 309 - DNA, 42 bp, Artificial
  Synthetic Polynucleotide
gtcgacttcggccaacgcgcggggtttttcttgatctacata

SEQ ID NO: 310 - DNA, 44 bp, Artificial
  Synthetic Polynucleotide
ctgtgtgattgcgttgcgctcactagagttgcttgatctacata

SEQ ID NO: 311 - DNA, 44 bp, Artificial
  Synthetic Polynucleotide
gcaattcacatattcctgattatcaaagtgtattgatctacata

SEQ ID NO: 312 - DNA, 42 bp, Artificial
  Synthetic Polynucleotide
ctaccatagtttgagtaacatttaaaatatttgatctacata

SEQ ID NO: 313 - DNA, 44 bp, Artificial
  Synthetic Polynucleotide
aagcctggtacgagccggaagcatagatgatgttgatctacata

SEQ ID NO: 314 - DNA, 44 bp, Artificial
  Synthetic Polynucleotide
agcaagcgtagggttgagtgttgtagggagccttgatctacata

SEQ ID NO: 315 - DNA, 44 bp, Artificial
  Synthetic Polynucleotide
tcaatatcgaacctcaaatatcaattccgaaattgatctacata

SEQ ID NO: 316 - DNA, 42 bp, Artificial
  Synthetic Polynucleotide
ctttagggcctgcaacagtgccaatacgtgttgatctacata

SEQ ID NO: 317 - DNA, 44 bp, Artificial
  Synthetic Polynucleotide
ctccaacgcagtgagacgggcaaccagctgcattgatctacata

SEQ ID NO: 318 - DNA, 42 bp, Artificial
  Synthetic Polynucleotide
tggaacaaccgcctggccctgaggcccgctttgatctacata

SEQ ID NO: 319 - DNA, 44 bp, Artificial
  Synthetic Polynucleotide
gcccgagagtccacgctggtttgcagctaactttgatctacata

SEQ ID NO: 320 - DNA, 44 bp, Artificial
  Synthetic Polynucleotide
tcggcaaatcctgtttgatggtggaccctcaattgatctacata

SEQ ID NO: 321 - DNA, 42 bp, Artificial
  Synthetic Polynucleotide
accttgcttggtcagttggcaaagagcggattgatctacata

SEQ ID NO: 322 - DNA, 44 bp, Artificial
  Synthetic Polynucleotide
agccagcaattgaggaaggttatcatcattttttgatctacata

SEQ ID NO: 323 - DNA, 44 bp, Artificial
  Synthetic Polynucleotide
ttaacaccagcactaacaactaatcgttattattgatctacata

SEQ ID NO: 324 - DNA, 42 bp, Artificial
  Synthetic Polynucleotide
cagaagattagataatacatttgtcgacaattgatctacata

SEQ ID NO: 325 - DNA, 42 bp, Artificial
  Synthetic Polynucleotide
aaagcactaaatcggaaccctaatccagttttgatctacata

SEQ ID NO: 326 - DNA, 44 bp, Artificial
  Synthetic Polynucleotide
cccgatttagagcttgacggggaaaaagaatattgatctacata

SEQ ID NO: 327 - DNA, 43 bp, Artificial
  Synthetic Polynucleotide
aacgtggcgagaaaggaagggaaaccagtaattgatctacata

SEQ ID NO: 328 - DNA, 42 bp, Artificial
  Synthetic Polynucleotide
taaaagggacattctggccaacaaagcatcttgatctacata

SEQ ID NO: 329 - DNA, 44 bp, Artificial
  Synthetic Polynucleotide
acccttctgacctgaaagcgtaagacgctgagttgatctacata

SEQ ID NO: 330 - DNA, 52 bp, Artificial
  Synthetic Polynucleotide
atgcagatacataacgggaatcgtcataaataaagcaaagttgatctacata

SEQ ID NO: 331 - DNA, 50 bp, Artificial
  Synthetic Polynucleotide
cgtttaccagacgacaaagaagttttgccataattcgattgatctacata

SEQ ID NO: 332 - DNA, 52 bp, Artificial
  Synthetic Polynucleotide
cgtagaaaatacataccgaggaaacgcaataagaagcgcattgatctacata

SEQ ID NO: 333 - DNA, 52 bp, Artificial
  Synthetic Polynucleotide
gtttattttgtcacaatcttaccgaagccctttaatatcattgatctacata

SEQ ID NO: 334 - DNA, 42 bp, Artificial
  Synthetic Polynucleotide
aacagttttgtaccaaaaacattttatttcttgatctacata

SEQ ID NO: 335 - DNA, 44 bp, Artificial
  Synthetic Polynucleotide
gatttagtcaataaagcctcagagaaccctcattgatctacata

SEQ ID NO: 336 - DNA, 44 bp, Artificial
  Synthetic Polynucleotide
aatggtcaacaggcaaggcaaagagtaatgtgttgatctacata

SEQ ID NO: 337 - DNA, 42 bp, Artificial
  Synthetic Polynucleotide
tttggggatagtagtagcattaaaaggccgttgatctacata

SEQ ID NO: 338 - DNA, 44 bp, Artificial
  Synthetic Polynucleotide
ccaatagctcatcgtaggaatcatggcatcaattgatctacata

SEQ ID NO: 339 - DNA, 44 bp, Artificial
  Synthetic Polynucleotide
tatccggtctcatcgagaacaagcgacaaaagttgatctacata

SEQ ID NO: 340 - DNA, 42 bp, Artificial
  Synthetic Polynucleotide
gcgaacctccaagaacgggtatgacaataattgatctacata

SEQ ID NO: 341 - DNA, 44 bp, Artificial
  Synthetic Polynucleotide
gccttaaaccaatcaataatcggcacgcgcctttgatctacata

SEQ ID NO: 342 - DNA, 44 bp, Artificial
  Synthetic Polynucleotide
aacaagagggataaaaatttttagcataaagcttgatctacata

SEQ ID NO: 343 - DNA, 42 bp, Artificial
  Synthetic Polynucleotide
gctatcagaaatgcaatgcctgaattagcattgatctacata

SEQ ID NO: 344 - DNA, 44 bp, Artificial
  Synthetic Polynucleotide
gagggtaggattcaaaagggtgagacatccaattgatctacata

SEQ ID NO: 345 - DNA, 44 bp, Artificial
  Synthetic Polynucleotide
caaccgtttcaaatcaccatcaattcgagccattgatctacata

SEQ ID NO: 346 - DNA, 42 bp, Artificial
  Synthetic Polynucleotide
catgtaatagaatataaagtaccaagccgtttgatctacata

SEQ ID NO: 347 - DNA, 44 bp, Artificial
  Synthetic Polynucleotide
aattgagaattctgtccagacgactaaaccaattgatctacata

SEQ ID NO: 348 - DNA, 44 bp, Artificial
  Synthetic Polynucleotide
agtataaagttcagctaatgcagatgtctttcttgatctacata

SEQ ID NO: 349 - DNA, 50 bp, Artificial
  Synthetic Polynucleotide
cccagcaggcgaaaaatcccttataaatcaagccggcgttgatctacata

SEQ ID NO: 350 - DNA, 52 bp, Artificial
  Synthetic Polynucleotide
tcaacagttgaaaggagcaaatgaaaaatctagagatagattgatctacata

SEQ ID NO: 351 - DNA, 44 bp, Artificial
  Synthetic Polynucleotide
ttaggattggctgagactcctcaataaccgatttgatctacata

SEQ ID NO: 352 - DNA, 44 bp, Artificial
  Synthetic Polynucleotide
gaccaactaatgccactacgaagggggtagcattgatctacata

SEQ ID NO: 353 - DNA, 42 bp, Artificial
  Synthetic Polynucleotide
gcgcagacaagaggcaaaagaatccctcagttgatctacata

SEQ ID NO: 354 - DNA, 44 bp, Artificial
  Synthetic Polynucleotide
gacctgctctttgacccccagcgagggagttattgatctacata

SEQ ID NO: 355 - DNA, 42 bp, Artificial
  Synthetic Polynucleotide
caccagaaaggttgaggcaggtcatgaaagttgatctacata

SEQ ID NO: 356 - DNA, 44 bp, Artificial
  Synthetic Polynucleotide
ccaccctctattcacaaacaaatacctgcctattgatctacata

SEQ ID NO: 357 - DNA, 44 bp, Artificial
  Synthetic Polynucleotide
gcctccctcagaatggaaagcgcagtaacagtttgatctacata

SEQ ID NO: 358 - DNA, 42 bp, Artificial
  Synthetic Polynucleotide
aaatcaccttccagtaagcgtcagtaataattgatctacata

SEQ ID NO: 359 - DNA, 44 bp, Artificial
  Synthetic Polynucleotide
gcaaggcctcaccagtagcaccatgggcttgattgatctacata

SEQ ID NO: 360 - DNA, 44 bp, Artificial
  Synthetic Polynucleotide
atccccctataccacattcaactagaaaaatcttgatctacata

SEQ ID NO: 361 - DNA, 42 bp, Artificial
  Synthetic Polynucleotide
aatactgcccaaaaggaattacgtggctcattgatctacata

SEQ ID NO: 362 - DNA, 44 bp, Artificial
  Synthetic Polynucleotide
aatagtaaacactatcataaccctcattgtgattgatctacata

SEQ ID NO: 363 - DNA, 42 bp, Artificial
  Synthetic Polynucleotide
atacccaacagtatgttagcaaattagagcttgatctacata

SEQ ID NO: 364 - DNA, 44 bp, Artificial
  Synthetic Polynucleotide
aaggaaacataaaggtggcaacattatcaccgttgatctacata

SEQ ID NO: 365 - DNA, 44 bp, Artificial
  Synthetic Polynucleotide
aagtaagcagacaccacggaataatattgacgttgatctacata

SEQ ID NO: 366 - DNA, 42 bp, Artificial
  Synthetic Polynucleotide
aatagctatcaatagaaaattcaacattcattgatctacata

SEQ ID NO: 367 - DNA, 44 bp, Artificial
  Synthetic Polynucleotide
agagagaaaaaaatgaaaatagcaagcaaactttgatctacata

SEQ ID NO: 368 - DNA, 44 bp, Artificial
  Synthetic Polynucleotide
taaatcgggattcccaattctgcgatataatgttgatctacata

SEQ ID NO: 369 - DNA, 42 bp, Artificial
  Synthetic Polynucleotide
aaattaagttgaccattagatacttttgcgttgatctacata

SEQ ID NO: 370 - DNA, 44 bp, Artificial
  Synthetic Polynucleotide
taaatcatataacctgtttagctaacctttaattgatctacata

SEQ ID NO: 371 - DNA, 42 bp, Artificial
  Synthetic Polynucleotide
ttttatttaagcaaatcagatattttttgtttgatctacata

SEQ ID NO: 372 - DNA, 44 bp, Artificial
  Synthetic Polynucleotide
gtaccgcaattctaagaacgcgagtattatttttgatctacata

SEQ ID NO: 373 - DNA, 44 bp, Artificial
  Synthetic Polynucleotide
cttatcattcccgacttgcgggagcctaatttttgatctacata

SEQ ID NO: 374 - DNA, 42 bp, Artificial
  Synthetic Polynucleotide
tgtagaaatcaagattagttgctcttaccattgatctacata

SEQ ID NO: 375 - DNA, 44 bp, Artificial
  Synthetic Polynucleotide
gtaataagttaggcagaggcatttatgatattttgatctacata

SEQ ID NO: 376 - DNA, 44 bp, Artificial
  Synthetic Polynucleotide
acaaacggaaaagccccaaaaacactggagcattgatctacata

SEQ ID NO: 377 - DNA, 42 bp, Artificial
  Synthetic Polynucleotide
gcgagtaaaaatatttaaattgttacaaagttgatctacata

SEQ ID NO: 378 - DNA, 44 bp, Artificial
  Synthetic Polynucleotide
tgtagccattaaaattcgcattaaatgccggattgatctacata

SEQ ID NO: 379 - DNA, 42 bp, Artificial
  Synthetic Polynucleotide
tataactaacaaagaacgcgagaacgccaattgatctacata

SEQ ID NO: 380 - DNA, 44 bp, Artificial
  Synthetic Polynucleotide
acctttttattttagttaatttcatagggcttttgatctacata

SEQ ID NO: 381 - DNA, 44 bp, Artificial
  Synthetic Polynucleotide
gaatttatttaatggtttgaaatattcttaccttgatctacata

SEQ ID NO: 382 - DNA, 42 bp, Artificial
  Synthetic Polynucleotide
cttagatttaaggcgttaaataaagcctgtttgatctacata

SEQ ID NO: 383 - DNA, 44 bp, Artificial
  Synthetic Polynucleotide
agaaaacaaagaagatgatgaaacaggctgcgttgatctacata

SEQ ID NO: 384 - DNA, 44 bp, Artificial
  Synthetic Polynucleotide
ttaatgaactagaggatccccggggggtaacgttgatctacata

SEQ ID NO: 385 - DNA, 42 bp, Artificial
  Synthetic Polynucleotide
ttccagtcgtaatcatggtcataaaaggggttgatctacata

SEQ ID NO: 386 - DNA, 44 bp, Artificial
  Synthetic Polynucleotide
cacattaaaattgttatccgctcatgcgggccttgatctacata

SEQ ID NO: 387 - DNA, 42 bp, Artificial
  Synthetic Polynucleotide
attatcattcaatataatcctgacaattacttgatctacata

SEQ ID NO: 388 - DNA, 44 bp, Artificial
  Synthetic Polynucleotide
gcggaacatctgaataatggaaggtacaaaatttgatctacata

SEQ ID NO: 389 - DNA, 44 bp, Artificial
  Synthetic Polynucleotide
attttaaaatcaaaattatttgcacggattcgttgatctacata

SEQ ID NO: 390 - DNA, 42 bp, Artificial
  Synthetic Polynucleotide
ctcgtattagaaattgcgtagatacagtacttgatctacata

SEQ ID NO: 391 - DNA, 43 bp, Artificial
  Synthetic Polynucleotide
agaaaggaacaactaaaggaattcaaaaaaattgatctacata

SEQ ID NO: 392 - DNA, 44 bp, Artificial
  Synthetic Polynucleotide
acaactttcaacagtttcagcggatgtatcggttgatctacata

SEQ ID NO: 393 - DNA, 44 bp, Artificial
  Synthetic Polynucleotide
ccaccctcattttcagggatagcaaccgtactttgatctacata

SEQ ID NO: 394 - DNA, 44 bp, Artificial
  Synthetic Polynucleotide
acggctacaaaaggagcctttaatgtgagaatttgatctacata

SEQ ID NO: 395 - DNA, 44 bp, Artificial
  Synthetic Polynucleotide
gcccgtatccggaataggtgtatcagcccaatttgatctacata

SEQ ID NO: 396 - DNA, 42 bp, Artificial
  Synthetic Polynucleotide
gttttaacttagtaccgccacccagagccattgatctacata

SEQ ID NO: 397 - DNA, 42 bp, Artificial
  Synthetic Polynucleotide
ttttcactcaaagggcgaaaaaccatcaccttgatctacata

SEQ ID NO: 398 - DNA, 52 bp, Artificial
  Synthetic Polynucleotide
agctgattgcccttcagagtccactattaaagggtgccgtttgatctacata

SEQ ID NO: 399 - DNA, 52 bp, Artificial
  Synthetic Polynucleotide
agattagagccgtcaaaaaacagaggtgaggcctattagtttgatctacata

SEQ ID NO: 400 - DNA, 43 bp, Artificial
  Synthetic Polynucleotide
caaatcaagttttttggggtcgaaacgtggattgatctacata

SEQ ID NO: 401 - DNA, 43 bp, Artificial
  Synthetic Polynucleotide
gcacagacaatatttttgaatggggtcagtattgatctacata

SEQ ID NO: 402 - DNA, 42 bp, Artificial
  Synthetic Polynucleotide
ctttaatgcgcgaactgatagccccaccagttgatctacata

SEQ ID NO: 403 - DNA, 40 bp, Artificial
  Synthetic Polynucleotide
ataagggaaccggatattcattacgtcaggacgttgggaa

SEQ ID NO: 404 - DNA, 38 bp, Artificial
  Synthetic Polynucleotide
ttgtgtcgtgacgagaaacaccaaatttcaactttaat

SEQ ID NO: 405 - DNA, 40 bp, Artificial
  Synthetic Polynucleotide
caccctcagaaaccatcgatagcattgagccatttgggaa

SEQ ID NO: 406 - DNA, 40 bp, Artificial
  Synthetic Polynucleotide
agccaccactgtagcgcgttttcaagggagggaaggtaaa

SEQ ID NO: 407 - DNA, 40 bp, Artificial
  Synthetic Polynucleotide
attaagtttaccgagctcgaattcgggaaacctgtcgtgc

SEQ ID NO: 408 - DNA, 38 bp, Artificial
  Synthetic Polynucleotide
gcgatcggcaattccacacaacaggtgcctaatgagtg

SEQ ID NO: 409 - DNA, 40 bp, Artificial
  Synthetic Polynucleotide
attcatttttgtttggattatactaagaaaccaccagaag

SEQ ID NO: 410 - DNA, 40 bp, Artificial
  Synthetic Polynucleotide
aacaataacgtaaaacagaaataaaaatcctttgcccgaa

SEQ ID NO: 411 - DNA, 48 bp, Artificial
  Synthetic Polynucleotide
tttatcaggacagcatcggaacgacaccaacctaaaacgaggtcaatc

SEQ ID NO: 412 - DNA, 44 bp, Artificial
  Synthetic Polynucleotide
tgacaactcgctgaggcttgcattataccaagcgcgatgataaa

SEQ ID NO: 413 - DNA, 48 bp, Artificial
  Synthetic Polynucleotide
gcggataacctattattctgaaacagacgattggccttgaagagccac

SEQ ID NO: 414 - DNA, 48 bp, Artificial
  Synthetic Polynucleotide
caggaggtggggtcagtgccttgagtctctgaatttaccgggaaccag

SEQ ID NO: 415 - DNA, 48 bp, Artificial
  Synthetic Polynucleotide
gtataagccaacccgtcggattctgacgacagtatcggccgcaaggcg

SEQ ID NO: 416 - DNA, 44 bp, Artificial
  Synthetic Polynucleotide
taaatcaaaataattcgcgtctcggaaaccaggcaaagggaagg

SEQ ID NO: 417 - DNA, 48 bp, Artificial
  Synthetic Polynucleotide
tcaaatataacctccggcttaggtaacaatttcatttgaaggcgaatt

SEQ ID NO: 418 - DNA, 48 bp, Artificial
  Synthetic Polynucleotide
gtgataaaaagacgctgagaagagataaccttgcttctgttcgggaga

SEQ ID NO: 419 - DNA, 32 bp, Artificial
  Synthetic Polynucleotide
aaggaattgcgaataataatttttgtcgctga

SEQ ID NO: 420 - DNA, 31 bp, Artificial
  Synthetic Polynucleotide
tcagcggagtgagaatagaaaggttttgcgg

SEQ ID NO: 421 - DNA, 32 bp, Artificial
  Synthetic Polynucleotide
tatgggattttgctaaacaactttcaacagtt

SEQ ID NO: 422 - DNA, 32 bp, Artificial
  Synthetic Polynucleotide
gaaaatctccaaaaaaaaggctccaaccatcg

SEQ ID NO: 423 - DNA, 32 bp, Artificial
  Synthetic Polynucleotide
ggtgtatcttgatataagtatagcgacagcat

SEQ ID NO: 424 - DNA, 32 bp, Artificial
  Synthetic Polynucleotide
tacgaaggcgccgacaatgacaacaaaaggag

SEQ ID NO: 425 - DNA, 32 bp, Artificial
  Synthetic Polynucleotide
aaagcgcaaaatcctcattaaagcggtcaatc

SEQ ID NO: 426 - DNA, 32 bp, Artificial
  Synthetic Polynucleotide
gcgtcagagcgacagaatcaagttgtcaggac

SEQ ID NO: 427 - DNA, 32 bp, Artificial
  Synthetic Polynucleotide
cggaataatataaaagaaacgcaaggaatcgt

SEQ ID NO: 428 - DNA, 30 bp, Artificial
  Synthetic Polynucleotide
agaaacgatttaagaaaagtaagcgaggaa

SEQ ID NO: 429 - DNA, 32 bp, Artificial
  Synthetic Polynucleotide
tgcgggagggcgttttagcgaacccaataaag

SEQ ID NO: 430 - DNA, 30 bp, Artificial
  Synthetic Polynucleotide
agaacaagcctaatttgccagttccaaata

SEQ ID NO: 431 - DNA, 32 bp, Artificial
  Synthetic Polynucleotide
aatgcagacgacaataaacaacatgtcattgc

SEQ ID NO: 432 - DNA, 30 bp, Artificial
  Synthetic Polynucleotide
tatttaactgtctttccttatcactcatcg

SEQ ID NO: 433 - DNA, 32 bp, Artificial
  Synthetic Polynucleotide
ttgaaataatcttctgacctaaatcaacccgt

SEQ ID NO: 434 - DNA, 30 bp, Artificial
  Synthetic Polynucleotide
ggcttaggttcttaccagtataaatcgcca

SEQ ID NO: 435 - DNA, 32 bp, Artificial
  Synthetic Polynucleotide
gtgagtgagaaacagtacataaatgcaaggcg

SEQ ID NO: 436 - DNA, 30 bp, Artificial
  Synthetic Polynucleotide
tattcatttcaatagtgaatttaaacctcc

SEQ ID NO: 437 - DNA, 32 bp, Artificial
  Synthetic Polynucleotide
tatttgcaggttagaacctaccatgggaaacc

SEQ ID NO: 438 - DNA, 30 bp, Artificial
  Synthetic Polynucleotide
ttctgaaaagcccaataggaaccacaaact

SEQ ID NO: 439 - DNA, 30 bp, Artificial
  Synthetic Polynucleotide
caccagaacggattcgcctgattggcgaat

SEQ ID NO: 440 - DNA, 32 bp, Artificial
  Synthetic Polynucleotide
caactaatctaaaatatctttagggagtccac

SEQ ID NO: 441 - DNA, 30 bp, Artificial
  Synthetic Polynucleotide
aaaaatctcgttattaattttaaaagaaac

SEQ ID NO: 442 - DNA, 30 bp, Artificial
  Synthetic Polynucleotide
ccaccctcgtaacagtgcccgtacctatta

SEQ ID NO: 443 - DNA, 30 bp, Artificial
  Synthetic Polynucleotide
atttgggaccggaaccgcctcccagagcca

SEQ ID NO: 444 - DNA, 30 bp, Artificial
  Synthetic Polynucleotide
acgcaatatattgacggaaattattgagcc

SEQ ID NO: 445 - DNA, 32 bp, Artificial
  Synthetic Polynucleotide
ttgagcgcaccctgaacaaagtcaagagctta

SEQ ID NO: 446 - DNA, 31 bp, Artificial
  Synthetic Polynucleotide
cctttaattgtatcggtttatcatgataccg

SEQ ID NO: 447 - DNA, 30 bp, Artificial
  Synthetic Polynucleotide
atagttgcaccaacctaaaacgctttgacc

SEQ ID NO: 448 - DNA, 30 bp, Artificial
  Synthetic Polynucleotide
tttagctaaccctcatatatttgattcaaa

SEQ ID NO: 449 - DNA, 30 bp, Artificial
  Synthetic Polynucleotide
agggtgaggaagattgtataagttaaaatt

SEQ ID NO: 450 - DNA, 30 bp, Artificial
  Synthetic Polynucleotide
cgcattagacgacagtatcggcgcaccgct

SEQ ID NO: 451 - DNA, 30 bp, Artificial
  Synthetic Polynucleotide
tctggtgtaccgagctcgaattaattgtta

SEQ ID NO: 452 - DNA, 30 bp, Artificial
  Synthetic Polynucleotide
tccgctcagctgattgcccttcgtccacgc

SEQ ID NO: 453 - DNA, 30 bp, Artificial
  Synthetic Polynucleotide
cccagcgaccggatattcattatgaataag

SEQ ID NO: 454 - DNA, 30 bp, Artificial
  Synthetic Polynucleotide
gcttgccatgcagatacataacacactatc

SEQ ID NO: 455 - DNA, 30 bp, Artificial
  Synthetic Polynucleotide
ataacccaagcaaagcggattgttcaaata

SEQ ID NO: 456 - DNA, 30 bp, Artificial
  Synthetic Polynucleotide
tcgcgttaacgagtagatttagataacctg

SEQ ID NO: 457 - DNA, 38 bp, Artificial
  Synthetic Polynucleotide
tagggttgagtgttgaacgtggactccaacgacctgaa

SEQ ID NO: 458 - DNA, 40 bp, Artificial
  Synthetic Polynucleotide
tcctgtttgatggtggaccatcacccaaatcacgagaaag

SEQ ID NO: 459 - DNA, 32 bp, Artificial
  Synthetic Polynucleotide
ataaatcaccgtctatcagggcgagacattct

SEQ ID NO: 460 - DNA, 31 bp, Artificial
  Synthetic Polynucleotide
acggggaaagccggcgaacgtggagtttttt

SEQ ID NO: 461 - DNA, 30 bp, Artificial
  Synthetic Polynucleotide
gaagggaaaccagtaataaaaggtggccca

SEQ ID NO: 462 - DNA, 32 bp, Artificial
  Synthetic Polynucleotide
ggccaacagagatagaacccttctgtcaaagg

SEQ ID NO: 463 - DNA, 40 bp, Artificial
  Synthetic Polynucleotide
atagataatacatttgtcaacagttgaaaggagcgcgaac

SEQ ID NO: 464 - DNA, 30 bp, Artificial
  Synthetic Polynucleotide
caaacaaaccctcaatcaatataaaaatac

SEQ ID NO: 465 - DNA, 40 bp, Artificial
  Synthetic Polynucleotide
aaatcctttgcccgaaaaagcatcaccttgctaaaacaga

SEQ ID NO: 466 - DNA, 30 bp, Artificial
  Synthetic Polynucleotide
tggtttgggtgccgtaaagcacagagcttg

SEQ ID NO: 467 - DNA, 31 bp, Artificial
  Synthetic Polynucleotide
agcgtaagaatacgtggcacagacaatattt

SEQ ID NO: 468 - DNA, 30 bp, Artificial
  Synthetic Polynucleotide
ttgaatggctattagtctttaatattgagg

SEQ ID NO: 469 - DNA, 32 bp, Artificial
  Synthetic Polynucleotide
tgatagccctaaaacatcgccattctggtcag

SEQ ID NO: 470 - DNA, 31 bp, Artificial
  Synthetic Polynucleotide
cgaacgaaccaccagcagaagatgaacctca

SEQ ID NO: 471 - DNA, 30 bp, Artificial
  Synthetic Polynucleotide
ggtgaggcggtcagtattaacacgcaaatg

SEQ ID NO: 472 - DNA, 32 bp, Artificial
  Synthetic Polynucleotide
ttgaggacgggagttaaaggccgcaacaacta

SEQ ID NO: 473 - DNA, 30 bp, Artificial
  Synthetic Polynucleotide
ttccattataaccgatatattcgtcacgtt

SEQ ID NO: 474 - DNA, 32 bp, Artificial
  Synthetic Polynucleotide
tctttccagacgttagtaaatgaatttagtac

SEQ ID NO: 475 - DNA, 31 bp, Artificial
  Synthetic Polynucleotide
atagttagcgtaacgatctaaagcagaaccg

SEQ ID NO: 476 - DNA, 32 bp, Artificial
  Synthetic Polynucleotide
acaacgcctgtagcattccacagaattttcag

SEQ ID NO: 477 - DNA, 44 bp, Artificial
  Synthetic Polynucleotide
gatcgtcgggtagcaacggctaccatgttacttagccaccgaac

SEQ ID NO: 478 - DNA, 48 bp, Artificial
  Synthetic Polynucleotide
cgccacccagtaccaggcggataagttccagtaagcgtcaagacgatt

SEQ ID NO: 479 - DNA, 30 bp, Artificial
  Synthetic Polynucleotide
ccaccctgagaaggattaggatatacagga

SEQ ID NO: 480 - DNA, 48 bp, Artificial
  Synthetic Polynucleotide
ggatagcacatgaaagtattaagaggggtcagtgccttgaagagccgc

SEQ ID NO: 481 - DNA, 48 bp, Artificial
  Synthetic Polynucleotide
cccacgcaaacgggtaaaatacgtaacaaagtacaacggagctgacct

SEQ ID NO: 482 - DNA, 32 bp, Artificial
  Synthetic Polynucleotide
ggcttgcataaagactttttcatgctgataaa

SEQ ID NO: 483 - DNA, 32 bp, Artificial
  Synthetic Polynucleotide
ttttaaatacctttaattgctccttcaaatgc

SEQ ID NO: 484 - DNA, 32 bp, Artificial
  Synthetic Polynucleotide
attgctgatttttgcggatggcttgagggtaa

SEQ ID NO: 485 - DNA, 30 bp, Artificial
  Synthetic Polynucleotide
aactgaactaatatcagagagatataaagg

SEQ ID NO: 486 - DNA, 32 bp, Artificial
  Synthetic Polynucleotide
aaaacagggttaagcccaataatagcagtatg

SEQ ID NO: 487 - DNA, 32 bp, Artificial
  Synthetic Polynucleotide
aaatagcagaaatagcaatagctaaagaactg

SEQ ID NO: 488 - DNA, 32 bp, Artificial
  Synthetic Polynucleotide
attctgcgttaattcgagcttcaatgactatt

SEQ ID NO: 489 - DNA, 30 bp, Artificial
  Synthetic Polynucleotide
gaagtttcagcaaactccaacagtgaccat

SEQ ID NO: 490 - DNA, 30 bp, Artificial
  Synthetic Polynucleotide
ggcaaagcataaagctaaatcgctattttt

SEQ ID NO: 491 - DNA, 32 bp, Artificial
  Synthetic Polynucleotide
tagttgctagaaggcttatccggtaacaatag

SEQ ID NO: 492 - DNA, 30 bp, Artificial
  Synthetic Polynucleotide
tcctgaataccgcgcccaatagtatcccat

SEQ ID NO: 493 - DNA, 32 bp, Artificial
  Synthetic Polynucleotide
ttccagagcaagccgtttttatttccaatcaa

SEQ ID NO: 494 - DNA, 32 bp, Artificial
  Synthetic Polynucleotide
gaaaaggtctttatttcaacgcaatcaaatca

SEQ ID NO: 495 - DNA, 32 bp, Artificial
  Synthetic Polynucleotide
tagcattatatgaccctgtaatactctagctg

SEQ ID NO: 496 - DNA, 32 bp, Artificial
  Synthetic Polynucleotide
aaaaacatacatccaataaatcattcaacatg

SEQ ID NO: 497 - DNA, 32 bp, Artificial
  Synthetic Polynucleotide
cctcagagaattagcaaaattaagtcccgact

SEQ ID NO: 498 - DNA, 30 bp, Artificial
  Synthetic Polynucleotide
gaacgcgagttttgaagccttaagagaatt

SEQ ID NO: 499 - DNA, 32 bp, Artificial
  Synthetic Polynucleotide
tcagatatattttgcacccagctaataacata

SEQ ID NO: 500 - DNA, 32 bp, Artificial
  Synthetic Polynucleotide
ggaatcattcttaccaacgctaacaaaaatga

SEQ ID NO: 501 - DNA, 32 bp, Artificial
  Synthetic Polynucleotide
atttttagatattttcatttgggggattccca

SEQ ID NO: 502 - DNA, 30 bp, Artificial
  Synthetic Polynucleotide
ggagaagcggcatcaattctactgtgtctg

SEQ ID NO: 503 - DNA, 30 bp, Artificial
  Synthetic Polynucleotide
gagagatctggagcaaacaagagctttcat

SEQ ID NO: 504 - DNA, 32 bp, Artificial
  Synthetic Polynucleotide
ataagtccgacaaaaggtaaagtaataaggcg

SEQ ID NO: 505 - DNA, 30 bp, Artificial
  Synthetic Polynucleotide
cctaatttcgagccagtaataacataatta

SEQ ID NO: 506 - DNA, 32 bp, Artificial
  Synthetic Polynucleotide
taatcggcaacgccaacatgtaatatatgcgt

SEQ ID NO: 507 - DNA, 32 bp, Artificial
  Synthetic Polynucleotide
ccatcaatcccggttgataatcaggctcattt

SEQ ID NO: 508 - DNA, 32 bp, Artificial
  Synthetic Polynucleotide
ataaattaatcgtaaaactagcataaaataat

SEQ ID NO: 509 - DNA, 32 bp, Artificial
  Synthetic Polynucleotide
gaacggtaatgccggagagggtaggttgtacc

SEQ ID NO: 510 - DNA, 32 bp, Artificial
  Synthetic Polynucleotide
ctgagagtctacaaaggctatcaggttcagct

SEQ ID NO: 511 - DNA, 30 bp, Artificial
  Synthetic Polynucleotide
ccagacgaacgcgcctgtttatcattctaa

SEQ ID NO: 512 - DNA, 32 bp, Artificial
  Synthetic Polynucleotide
aaagtacctgaacaagaaaaataacaagcaaa

SEQ ID NO: 513 - DNA, 32 bp, Artificial
  Synthetic Polynucleotide
aggcattttacgagcatgtagaaatcatcgta

SEQ ID NO: 514 - DNA, 32 bp, Artificial
  Synthetic Polynucleotide
caaaaacagaaaggccggagacagggataaaa

SEQ ID NO: 515 - DNA, 30 bp, Artificial
  Synthetic Polynucleotide
atatgtacatgatattcaaccgtttttgcg

SEQ ID NO: 516 - DNA, 44 bp, Artificial
  Synthetic Polynucleotide
caacattccgtgggaacaaacgattacgccagctggcgggtaac

SEQ ID NO: 517 - DNA, 48 bp, Artificial
  Synthetic Polynucleotide
ttaaataaaaactttttcaaatattaaatcgtcgctattaaacaattt

SEQ ID NO: 518 - DNA, 30 bp, Artificial
  Synthetic Polynucleotide
ctagaaacaaatccaatcgcaaaatccttg

SEQ ID NO: 519 - DNA, 48 bp, Artificial
  Synthetic Polynucleotide
tatacaaattgggttatataactaaagacgctgagaagagtcaattac

SEQ ID NO: 520 - DNA, 48 bp, Artificial
  Synthetic Polynucleotide
tttaaccatcgtaaccgtgcatctgcgccattcgccattctgcctgca

SEQ ID NO: 521 - DNA, 32 bp, Artificial
  Synthetic Polynucleotide
tcgcgtctgggataggtcacgttgtgggaagg

SEQ ID NO: 522 - DNA, 32 bp, Artificial
  Synthetic Polynucleotide
accgtaatggccttcctgtagccagaatcgat

SEQ ID NO: 523 - DNA, 32 bp, Artificial
  Synthetic Polynucleotide
cggattctaaatgtgagcgagtaattaatggt

SEQ ID NO: 524 - DNA, 30 bp, Artificial
  Synthetic Polynucleotide
ttaatttcccgaccgtgtgataaattctgt

SEQ ID NO: 525 - DNA, 32 bp, Artificial
  Synthetic Polynucleotide
acgcgagagaataaacaccggaatgagaatat

SEQ ID NO: 526 - DNA, 32 bp, Artificial
  Synthetic Polynucleotide
tgctgatgaagcctgtttagtatcttaggcag

SEQ ID NO: 527 - DNA, 32 bp, Artificial
  Synthetic Polynucleotide
gaggggacaatttttgttaaatcaaaaagccc

SEQ ID NO: 528 - DNA, 30 bp, Artificial
  Synthetic Polynucleotide
tgggcgcaataggaacgccatcagtcaatc

SEQ ID NO: 529 - DNA, 30 bp, Artificial
  Synthetic Polynucleotide
aaaacataaacatcaagaaaacagatgaat

SEQ ID NO: 530 - DNA, 32 bp, Artificial
  Synthetic Polynucleotide
gcgatcggttgtaaaacgacggccgggtgcct

SEQ ID NO: 531 - DNA, 32 bp, Artificial
  Synthetic Polynucleotide
tcacgacgtgcgggcctcttcgctgcggattg

SEQ ID NO: 532 - DNA, 32 bp, Artificial
  Synthetic Polynucleotide
attaagttgaaagggggatgtgctcaatatat

SEQ ID NO: 533 - DNA, 30 bp, Artificial
  Synthetic Polynucleotide
ttttaatgataaccttgcttctgattttag

SEQ ID NO: 534 - DNA, 32 bp, Artificial
  Synthetic Polynucleotide
ttacatttattaattttcccttaggacaaaga

SEQ ID NO: 535 - DNA, 32 bp, Artificial
  Synthetic Polynucleotide
gatgaaacagcgatagcttagatttatgtaaa

SEQ ID NO: 536 - DNA, 32 bp, Artificial
  Synthetic Polynucleotide
tccccgggccggaaaccaggcaaagccagttt

SEQ ID NO: 537 - DNA, 30 bp, Artificial
  Synthetic Polynucleotide
agcttgcaaggctgcgcaactgtgtgtaga

SEQ ID NO: 538 - DNA, 30 bp, Artificial
  Synthetic Polynucleotide
atacagtagatgatggcaattcagacttta

SEQ ID NO: 539 - DNA, 32 bp, Artificial
  Synthetic Polynucleotide
aatgagtgggagaggcggtttgcgaatccctt

SEQ ID NO: 540 - DNA, 32 bp, Artificial
  Synthetic Polynucleotide
cggaacgaaccctcagcagcgaaaccggaata

SEQ ID NO: 541 - DNA, 30 bp, Artificial
  Synthetic Polynucleotide
cgagagggaccgtactcaggaggttttctg

SEQ ID NO: 542 - DNA, 32 bp, Artificial
  Synthetic Polynucleotide
ttttgctctcagaaccgccaccctttttgtcg

SEQ ID NO: 543 - DNA, 32 bp, Artificial
  Synthetic Polynucleotide
ctcctcaacagagccaccaccctccagccctc

SEQ ID NO: 544 - DNA, 32 bp, Artificial
  Synthetic Polynucleotide
acgcgcggagctaactcacattaatttcccag

SEQ ID NO: 545 - DNA, 32 bp, Artificial
  Synthetic Polynucleotide
tgtcgtgctgcccgctttccagtcatcaaaat

SEQ ID NO: 546 - DNA, 30 bp, Artificial
  Synthetic Polynucleotide
aatggaagcgtaaaacagaaatattacctt

SEQ ID NO: 547 - DNA, 32 bp, Artificial
  Synthetic Polynucleotide
aatcctgatttcaggtttaacgtcaaaattaa

SEQ ID NO: 548 - DNA, 32 bp, Artificial
  Synthetic Polynucleotide
tgattatcaacagtaccttttacaaagaagat

SEQ ID NO: 549 - DNA, 32 bp, Artificial
  Synthetic Polynucleotide
cgggcaacacaattccacacaacactagagga

SEQ ID NO: 550 - DNA, 30 bp, Artificial
  Synthetic Polynucleotide
cgccagggaaagtgtaaagcctgagtgcca

SEQ ID NO: 551 - DNA, 32 bp, Artificial
  Synthetic Polynucleotide
gcgaaaaaaaagaatagcccgagaatcggcca

SEQ ID NO: 552 - DNA, 32 bp, Artificial
  Synthetic Polynucleotide
tattaaagttccagtttggaacaaagcactaa

SEQ ID NO: 553 - DNA, 30 bp, Artificial
  Synthetic Polynucleotide
aaggttatagattagagccgtcatctgaat

SEQ ID NO: 554 - DNA, 32 bp, Artificial
  Synthetic Polynucleotide
ttggcaaaaggatttagaagtattatcaatat

SEQ ID NO: 555 - DNA, 32 bp, Artificial
  Synthetic Polynucleotide
aatatcaattcgacaactcgtattcatattcc

SEQ ID NO: 556 - DNA, 32 bp, Artificial
  Synthetic Polynucleotide
ggggtcgaccccagcaggcgaaaacagtgaga

SEQ ID NO: 557 - DNA, 30 bp, Artificial
  Synthetic Polynucleotide
ctacgtgattccgaaatcggcaatattggg

SEQ ID NO: 558 - DNA, 30 bp, Artificial
  Synthetic Polynucleotide
gtgtactcgccagcattgacagcgtttgcc

SEQ ID NO: 559 - DNA, 32 bp, Artificial
  Synthetic Polynucleotide
ttgtgtcgtgaacggtgtacagactaatttca

SEQ ID NO: 560 - DNA, 32 bp, Artificial
  Synthetic Polynucleotide
aggacagaaaatccgcgacctgctcagaggct

SEQ ID NO: 561 - DNA, 32 bp, Artificial
  Synthetic Polynucleotide
ataagggaggaacgaggcgcagaccagaatgg

SEQ ID NO: 562 - DNA, 30 bp, Artificial
  Synthetic Polynucleotide
aaacaaatgtctctgaatttaccgtgccgt

SEQ ID NO: 563 - DNA, 32 bp, Artificial
  Synthetic Polynucleotide
ggcaggtctacatggcttttgatgtagcgggg

SEQ ID NO: 564 - DNA, 32 bp, Artificial
  Synthetic Polynucleotide
agagccgcggtaataagttttaacggctgaga

SEQ ID NO: 565 - DNA, 32 bp, Artificial
  Synthetic Polynucleotide
tgacaagaattataccaagcgcgaaatgccac

SEQ ID NO: 566 - DNA, 30 bp, Artificial
  Synthetic Polynucleotide
ataggctggatttgtatcatcgcaggaagt

SEQ ID NO: 567 - DNA, 30 bp, Artificial
  Synthetic Polynucleotide
atctttttaccattagcaaggccaaagaca

SEQ ID NO: 568 - DNA, 32 bp, Artificial
  Synthetic Polynucleotide
actttaatgaacaacattattacaaaaagaag

SEQ ID NO: 569 - DNA, 32 bp, Artificial
  Synthetic Polynucleotide
aactaacgcattgtgaattacctttttgaaag

SEQ ID NO: 570 - DNA, 32 bp, Artificial
  Synthetic Polynucleotide
gttgggaactggctcattataccatgccttta

SEQ ID NO: 571 - DNA, 30 bp, Artificial
  Synthetic Polynucleotide
aatcagtactgtagcgcgttttctattcac

SEQ ID NO: 572 - DNA, 32 bp, Artificial
  Synthetic Polynucleotide
tcaccaatatagcccccttattaggaggttga

SEQ ID NO: 573 - DNA, 32 bp, Artificial
  Synthetic Polynucleotide
agcaccatcataatcaaaatcaccccaccacc

SEQ ID NO: 574 - DNA, 32 bp, Artificial
  Synthetic Polynucleotide
ttcaactactgacgagaaacaccaagtaatct

SEQ ID NO: 575 - DNA, 30 bp, Artificial
  Synthetic Polynucleotide
agattcatgggcttgagatggttcaggcgc

SEQ ID NO: 576 - DNA, 38 bp, Artificial
  Synthetic Polynucleotide
aatgtttagactggattcattgaatccccctttgataa

SEQ ID NO: 577 - DNA, 40 bp, Artificial
  Synthetic Polynucleotide
atcaatagaaaattcacgtagaaaatacatacaacccaca

SEQ ID NO: 578 - DNA, 30 bp, Artificial
  Synthetic Polynucleotide
aaagggcaagactccttattacagagcaag

SEQ ID NO: 579 - DNA, 40 bp, Artificial
  Synthetic Polynucleotide
agggagggaaggtaaaataacggaatacccaatcttaccg

SEQ ID NO: 580 - DNA, 40 bp, Artificial
  Synthetic Polynucleotide
gataaaaaccaaaataaatcaggtctttacccagcgaacc

SEQ ID NO: 581 - DNA, 32 bp, Artificial
  Synthetic Polynucleotide
ttttgccagttcagaaaacgagaagtcaggat

SEQ ID NO: 582 - DNA, 32 bp, Artificial
  Synthetic Polynucleotide
tttaaacagagggggtaatagtaaataaaacg

SEQ ID NO: 583 - DNA, 32 bp, Artificial
  Synthetic Polynucleotide
cataaatatagcgtccaatactgcagacacca

SEQ ID NO: 584 - DNA, 30 bp, Artificial
  Synthetic Polynucleotide
tggcaacagtttattttgtcacagcaccgt

SEQ ID NO: 585 - DNA, 32 bp, Artificial
  Synthetic Polynucleotide
ttagcaaatatggtttaccagcgccggaaacg

SEQ ID NO: 586 - DNA, 32 bp, Artificial
  Synthetic Polynucleotide
gcatgattgacattcaaccgattgtcaccagt

SEQ ID NO: 587 - DNA, 32 bp, Artificial
  Synthetic Polynucleotide
atagtcagtcgtttaccagacgacataccaca

SEQ ID NO: 588 - DNA, 30 bp, Artificial
  Synthetic Polynucleotide
aaatcaaagcgagaggcttttgcggtagaa

SEQ ID NO: 589 - DNA, 30 bp, Artificial
  Synthetic Polynucleotide
gaggtcaatataatgctgtagcacaggcaa

SEQ ID NO: 590 - DNA, 32 bp, Artificial
  Synthetic Polynucleotide
agaattgagaagcgcattagacggatcaagat

SEQ ID NO: 591 - DNA, 30 bp, Artificial
  Synthetic Polynucleotide
aaacaatgcctttacagagagacaatttta

SEQ ID NO: 592 - DNA, 32 bp, Artificial
  Synthetic Polynucleotide
aagcccttttttttgtttaacgtcgagcgtct

SEQ ID NO: 593 - DNA, 32 bp, Artificial
  Synthetic Polynucleotide
agaccggaattccatataacagttcgcgagct

SEQ ID NO: 594 - DNA, 32 bp, Artificial
  Synthetic Polynucleotide
tagagagtatgcaactaaagtacgaatagtag

SEQ ID NO: 595 - DNA, 40 bp, Artificial; identical to SEQ ID NO: 403
  Synthetic Polynucleotide

SEQ ID NO: 596 - DNA, 38 bp, Artificial; identical to SEQ ID NO: 404
  Synthetic Polynucleotide

SEQ ID NO: 597 - DNA, 40 bp, Artificial; identical to SEQ ID NO: 405
  Synthetic Polynucleotide

SEQ ID NO: 598 - DNA, 40 bp, Artificial; identical to SEQ ID NO: 406
  Synthetic Polynucleotide

SEQ ID NO: 599 - DNA, 40 bp, Artificial; identical to SEQ ID NO: 407
  Synthetic Polynucleotide

SEQ ID NO: 600 - DNA, 38 bp, Artificial; identical to SEQ ID NO: 408
  Synthetic Polynucleotide

SEQ ID NO: 601 - DNA, 40 bp, Artificial; identical to SEQ ID NO: 409
  Synthetic Polynucleotide

SEQ ID NO: 602 - DNA, 40 bp, Artificial; identical to SEQ ID NO: 410
  Synthetic Polynucleotide

SEQ ID NO: 603 - DNA, 32 bp, Artificial; identical to SEQ ID NO: 423
  Synthetic Polynucleotide

SEQ ID NO: 604 - DNA, 32 bp, Artificial; identical to SEQ ID NO: 429
  Synthetic Polynucleotide

SEQ ID NO: 605 - DNA, 32 bp, Artificial; identical to SEQ ID NO: 431
  Synthetic Polynucleotide

SEQ ID NO: 606 - DNA, 32 bp, Artificial; identical to SEQ ID NO: 433
  Synthetic Polynucleotide

SEQ ID NO: 607 - DNA, 32 bp, Artificial; identical to SEQ ID NO: 435
  Synthetic Polynucleotide

SEQ ID NO: 608 - DNA, 32 bp, Artificial; identical to SEQ ID NO: 437
  Synthetic Polynucleotide

SEQ ID NO: 609 - DNA, 32 bp, Artificial; identical to SEQ ID NO: 440
  Synthetic Polynucleotide

SEQ ID NO: 610 - DNA, 32 bp, Artificial; identical to SEQ ID NO: 425
  Synthetic Polynucleotide

SEQ ID NO: 611 - DNA, 32 bp, Artificial; identical to SEQ ID NO: 426
  Synthetic Polynucleotide

SEQ ID NO: 612 - DNA, 32 bp, Artificial; identical to SEQ ID NO: 427
  Synthetic Polynucleotide

SEQ ID NO: 613 - DNA, 32 bp, Artificial; identical to SEQ ID NO: 445
  Synthetic Polynucleotide

SEQ ID NO: 614 - DNA, 30 bp, Artificial; identical to SEQ ID NO: 464
  Synthetic Polynucleotide

SEQ ID NO: 615 - DNA, 40 bp, Artificial; identical to SEQ ID NO: 465
  Synthetic Polynucleotide

SEQ ID NO: 616 - DNA, 32 bp, Artificial; identical to SEQ ID NO: 419
  Synthetic Polynucleotide

SEQ ID NO: 617 - DNA, 31 bp, Artificial; identical to SEQ ID NO: 420
  Synthetic Polynucleotide

SEQ ID NO: 618 - DNA, 32 bp, Artificial; identical to SEQ ID NO: 422
  Synthetic Polynucleotide

SEQ ID NO: 619 - DNA, 32 bp, Artificial; identical to SEQ ID NO: 472
  Synthetic Polynucleotide

SEQ ID NO: 620 - DNA, 32 bp, Artificial; identical to SEQ ID NO: 424
  Synthetic Polynucleotide

SEQ ID NO: 621 - DNA, 30 bp, Artificial; identical to SEQ ID NO: 473
  Synthetic Polynucleotide

SEQ ID NO: 622 - DNA, 40 bp, Artificial; identical to SEQ ID NO: 463
  Synthetic Polynucleotide

SEQ ID NO: 623 - DNA, 30 bp, Artificial; identical to SEQ ID NO: 468
  Synthetic Polynucleotide

SEQ ID NO: 624 - DNA, 32 bp, Artificial; identical to SEQ ID NO: 469
  Synthetic Polynucleotide

SEQ ID NO: 625 - DNA, 31 bp, Artificial; identical to SEQ ID NO: 470
  Synthetic Polynucleotide

SEQ ID NO: 626 - DNA, 30 bp, Artificial; identical to SEQ ID NO: 447
  Synthetic Polynucleotide

SEQ ID NO: 627 - DNA, 30 bp, Artificial; identical to SEQ ID NO: 448
  Synthetic Polynucleotide

SEQ ID NO: 628 - DNA, 30 bp, Artificial; identical to SEQ ID NO: 449
  Synthetic Polynucleotide

SEQ ID NO: 629 - DNA, 30 bp, Artificial; identical to SEQ ID NO: 450
  Synthetic Polynucleotide

SEQ ID NO: 630 - DNA, 30 bp, Artificial; identical to SEQ ID NO: 451
  Synthetic Polynucleotide

SEQ ID NO: 631 - DNA, 30 bp, Artificial; identical to SEQ ID NO: 452
  Synthetic Polynucleotide

SEQ ID NO: 632 - DNA, 30 bp, Artificial; identical to SEQ ID NO: 453
  Synthetic Polynucleotide

SEQ ID NO: 633 - DNA, 30 bp, Artificial; identical to SEQ ID NO: 454
  Synthetic Polynucleotide

SEQ ID NO: 634 - DNA, 30 bp, Artificial; identical to SEQ ID NO: 455
  Synthetic Polynucleotide

SEQ ID NO: 635 - DNA, 30 bp, Artificial; identical to SEQ ID NO: 456
  Synthetic Polynucleotide

SEQ ID NO: 636 - DNA, 32 bp, Artificial; identical to SEQ ID NO: 474
  Synthetic Polynucleotide

SEQ ID NO: 637 - DNA, 31 bp, Artificial; identical to SEQ ID NO: 475
  Synthetic Polynucleotide

SEQ ID NO: 638 - DNA, 32 bp, Artificial; identical to SEQ ID NO: 476
  Synthetic Polynucleotide

SEQ ID NO: 639 - DNA, 30 bp, Artificial; identical to SEQ ID NO: 428
  Synthetic Polynucleotide

SEQ ID NO: 640 - DNA, 30 bp, Artificial; identical to SEQ ID NO: 430
  Synthetic Polynucleotide

SEQ ID NO: 641 - DNA, 30 bp, Artificial; identical to SEQ ID NO: 432
  Synthetic Polynucleotide

SEQ ID NO: 642 - DNA, 30 bp, Artificial; identical to SEQ ID NO: 434
  Synthetic Polynucleotide

SEQ ID NO: 643 - DNA, 30 bp, Artificial; identical to SEQ ID NO: 436
  Synthetic Polynucleotide

SEQ ID NO: 644 - DNA, 30 bp, Artificial; identical to SEQ ID NO: 541
  Synthetic Polynucleotide

SEQ ID NO: 645 - DNA, 32 bp, Artificial; identical to SEQ ID NO: 542
  Synthetic Polynucleotide

SEQ ID NO: 646 - DNA, 32 bp, Artificial; identical to SEQ ID NO: 543
  Synthetic Polynucleotide

SEQ ID NO: 647 - DNA, 30 bp, Artificial; identical to SEQ ID NO: 438
  Synthetic Polynucleotide

SEQ ID NO: 648 - DNA, 30 bp, Artificial; identical to SEQ ID NO: 439
  Synthetic Polynucleotide

SEQ ID NO: 649 - DNA, 30 bp, Artificial; identical to SEQ ID NO: 441
  Synthetic Polynucleotide

SEQ ID NO: 650 - DNA, 30 bp, Artificial; identical to SEQ ID NO: 442
  Synthetic Polynucleotide

SEQ ID NO: 651 - DNA, 30 bp, Artificial; identical to SEQ ID NO: 443
  Synthetic Polynucleotide

SEQ ID NO: 652 - DNA, 30 bp, Artificial; identical to SEQ ID NO: 444
  Synthetic Polynucleotide

SEQ ID NO: 653 - DNA, 30 bp, Artificial; identical to SEQ ID NO: 466
  Synthetic Polynucleotide

SEQ ID NO: 654 - DNA, 40 bp, Artificial; identical to SEQ ID NO: 458
  Synthetic Polynucleotide

SEQ ID NO: 655 - DNA, 32 bp, Artificial; identical to SEQ ID NO: 459
  Synthetic Polynucleotide

SEQ ID NO: 656 - DNA, 31 bp, Artificial; identical to SEQ ID NO: 460
  Synthetic Polynucleotide

SEQ ID NO: 657 - DNA, 30 bp, Artificial; identical to SEQ ID NO: 461
  Synthetic Polynucleotide

SEQ ID NO: 658 - DNA, 32 bp, Artificial; identical to SEQ ID NO: 462
  Synthetic Polynucleotide

SEQ ID NO: 659 - DNA, 32 bp, Artificial; identical to SEQ ID NO: 421
  Synthetic Polynucleotide

SEQ ID NO: 660 - DNA, 31 bp, Artificial; identical to SEQ ID NO: 446
  Synthetic Polynucleotide

SEQ ID NO: 661 - DNA, 31 bp, Artificial; identical to SEQ ID NO: 467
  Synthetic Polynucleotide

SEQ ID NO: 662 - DNA, 30 bp, Artificial; identical to SEQ ID NO: 471
  Synthetic Polynucleotide

SEQ ID NO: 663 - DNA, 38 bp, Artificial; identical to SEQ ID NO: 457
  Synthetic Polynucleotide

SEQ ID NO: 664 - DNA, 44 bp, Artificial; identical to SEQ ID NO: 477
  Synthetic Polynucleotide

SEQ ID NO: 665 - DNA, 48 bp, Artificial; identical to SEQ ID NO: 478
  Synthetic Polynucleotide

SEQ ID NO: 666 - DNA, 30 bp, Artificial; identical to SEQ ID NO: 479
  Synthetic Polynucleotide

SEQ ID NO: 667 - DNA, 48 bp, Artificial; identical to SEQ ID NO: 480
  Synthetic Polynucleotide

SEQ ID NO: 668 - DNA, 48 bp, Artificial; identical to SEQ ID NO: 481
  Synthetic Polynucleotide

SEQ ID NO: 669 - DNA, 32 bp, Artificial; identical to SEQ ID NO: 482
  Synthetic Polynucleotide

SEQ ID NO: 670 - DNA, 32 bp, Artificial; identical to SEQ ID NO: 483
  Synthetic Polynucleotide

SEQ ID NO: 671 - DNA, 32 bp, Artificial; identical to SEQ ID NO: 484
  Synthetic Polynucleotide

SEQ ID NO: 672 - DNA, 30 bp, Artificial; identical to SEQ ID NO: 485
  Synthetic Polynucleotide

SEQ ID NO: 673 - DNA, 32 bp, Artificial; identical to SEQ ID NO: 486
  Synthetic Polynucleotide

SEQ ID NO: 674 - DNA, 32 bp, Artificial; identical to SEQ ID NO: 487
  Synthetic Polynucleotide

SEQ ID NO: 675 - DNA, 32 bp, Artificial; identical to SEQ ID NO: 488
  Synthetic Polynucleotide

SEQ ID NO: 676 - DNA, 30 bp, Artificial; identical to SEQ ID NO: 489
  Synthetic Polynucleotide

SEQ ID NO: 677 - DNA, 30 bp, Artificial; identical to SEQ ID NO: 490
  Synthetic Polynucleotide

SEQ ID NO: 678 - DNA, 32 bp, Artificial; identical to SEQ ID NO: 491
  Synthetic Polynucleotide

SEQ ID NO: 679 - DNA, 30 bp, Artificial; identical to SEQ ID NO: 492
  Synthetic Polynucleotide

SEQ ID NO: 680 - DNA, 32 bp, Artificial; identical to SEQ ID NO: 493
  Synthetic Polynucleotide

SEQ ID NO: 681 - DNA, 32 bp, Artificial; identical to SEQ ID NO: 494
  Synthetic Polynucleotide

SEQ ID NO: 682 - DNA, 32 bp, Artificial; identical to SEQ ID NO: 495
  Synthetic Polynucleotide

SEQ ID NO: 683 - DNA, 32 bp, Artificial; identical to SEQ ID NO: 496
  Synthetic Polynucleotide

SEQ ID NO: 684 - DNA, 32 bp, Artificial; identical to SEQ ID NO: 497
  Synthetic Polynucleotide

SEQ ID NO: 685 - DNA, 30 bp, Artificial; identical to SEQ ID NO: 498
  Synthetic Polynucleotide

SEQ ID NO: 686 - DNA, 32 bp, Artificial; identical to SEQ ID NO: 499
  Synthetic Polynucleotide

SEQ ID NO: 687 - DNA, 32 bp, Artificial; identical to SEQ ID NO: 500
  Synthetic Polynucleotide

SEQ ID NO: 688 - DNA, 32 bp, Artificial; identical to SEQ ID NO: 501
  Synthetic Polynucleotide

SEQ ID NO: 689 - DNA, 30 bp, Artificial; identical to SEQ ID NO: 502
  Synthetic Polynucleotide

SEQ ID NO: 690 - DNA, 30 bp, Artificial; identical to SEQ ID NO: 503
  Synthetic Polynucleotide

SEQ ID NO: 691 - DNA, 32 bp, Artificial; identical to SEQ ID NO: 504
  Synthetic Polynucleotide

SEQ ID NO: 692 - DNA, 30 bp, Artificial; identical to SEQ ID NO: 505
  Synthetic Polynucleotide

SEQ ID NO: 693 - DNA, 32 bp, Artificial; identical to SEQ ID NO: 506
  Synthetic Polynucleotide

SEQ ID NO: 694 - DNA, 32 bp, Artificial; identical to SEQ ID NO: 507
  Synthetic Polynucleotide

SEQ ID NO: 695 - DNA, 32 bp, Artificial; identical to SEQ ID NO: 508
  Synthetic Polynucleotide

SEQ ID NO: 696 - DNA, 32 bp, Artificial; identical to SEQ ID NO: 509
  Synthetic Polynucleotide

SEQ ID NO: 697 - DNA, 32 bp, Artificial; identical to SEQ ID NO: 510
  Synthetic Polynucleotide

SEQ ID NO: 698 - DNA, 30 bp, Artificial; identical to SEQ ID NO: 511
  Synthetic Polynucleotide

SEQ ID NO: 699 - DNA, 32 bp, Artificial; identical to SEQ ID NO: 512
  Synthetic Polynucleotide

SEQ ID NO: 700 - DNA, 32 bp, Artificial; identical to SEQ ID NO: 513
  Synthetic Polynucleotide

SEQ ID NO: 701 - DNA, 32 bp, Artificial; identical to SEQ ID NO: 514
  Synthetic Polynucleotide

SEQ ID NO: 702 - DNA, 30 bp, Artificial; identical to SEQ ID NO: 515
  Synthetic Polynucleotide

SEQ ID NO: 703 - DNA, 44 bp, Artificial; identical to SEQ ID NO: 516
  Synthetic Polynucleotide

SEQ ID NO: 704 - DNA, 48 bp, Artificial; identical to SEQ ID NO: 517
  Synthetic Polynucleotide

SEQ ID NO: 705 - DNA, 30 bp, Artificial; identical to SEQ ID NO: 518
  Synthetic Polynucleotide

SEQ ID NO: 706 - DNA, 48 bp, Artificial; identical to SEQ ID NO: 519
  Synthetic Polynucleotide

SEQ ID NO: 707 - DNA, 48 bp, Artificial; identical to SEQ ID NO: 520
  Synthetic Polynucleotide

SEQ ID NO: 708 - DNA, 32 bp, Artificial; identical to SEQ ID NO: 521
  Synthetic Polynucleotide

SEQ ID NO: 709 - DNA, 32 bp, Artificial; identical to SEQ ID NO: 522
  Synthetic Polynucleotide

SEQ ID NO: 710 - DNA, 32 bp, Artificial; identical to SEQ ID NO: 523
  Synthetic Polynucleotide

SEQ ID NO: 711 - DNA, 30 bp, Artificial; identical to SEQ ID NO: 524
  Synthetic Polynucleotide

SEQ ID NO: 712 - DNA, 32 bp, Artificial; identical to SEQ ID NO: 525
  Synthetic Polynucleotide

SEQ ID NO: 713 - DNA, 32 bp, Artificial; identical to SEQ ID NO: 526
  Synthetic Polynucleotide

SEQ ID NO: 714 - DNA, 32 bp, Artificial; identical to SEQ ID NO: 527
  Synthetic Polynucleotide

SEQ ID NO: 715 - DNA, 30 bp, Artificial; identical to SEQ ID NO: 528
  Synthetic Polynucleotide

SEQ ID NO: 716 - DNA, 30 bp, Artificial; identical to SEQ ID NO: 529
  Synthetic Polynucleotide

SEQ ID NO: 717 - DNA, 32 bp, Artificial; identical to SEQ ID NO: 530
  Synthetic Polynucleotide

SEQ ID NO: 718 - DNA, 32 bp, Artificial; identical to SEQ ID NO: 531
  Synthetic Polynucleotide

SEQ ID NO: 719 - DNA, 32 bp, Artificial; identical to SEQ ID NO: 532
  Synthetic Polynucleotide

SEQ ID NO: 720 - DNA, 30 bp, Artificial; identical to SEQ ID NO: 533
  Synthetic Polynucleotide

SEQ ID NO: 721 - DNA, 32 bp, Artificial; identical to SEQ ID NO: 534
  Synthetic Polynucleotide

SEQ ID NO: 722 - DNA, 32 bp, Artificial; identical to SEQ ID NO: 535
  Synthetic Polynucleotide

SEQ ID NO: 723 - DNA, 32 bp, Artificial; identical to SEQ ID NO: 536
  Synthetic Polynucleotide

SEQ ID NO: 724 - DNA, 30 bp, Artificial; identical to SEQ ID NO: 537
  Synthetic Polynucleotide

SEQ ID NO: 725 - DNA, 30 bp, Artificial; identical to SEQ ID NO: 538
  Synthetic Polynucleotide

SEQ ID NO: 726 - DNA, 32 bp, Artificial; identical to SEQ ID NO: 539
  Synthetic Polynucleotide

SEQ ID NO: 727 - DNA, 32 bp, Artificial; identical to SEQ ID NO: 540
  Synthetic Polynucleotide

SEQ ID NO: 728 - DNA, 32 bp, Artificial; identical to SEQ ID NO: 544
  Synthetic Polynucleotide

SEQ ID NO: 729 - DNA, 32 bp, Artificial; identical to SEQ ID NO: 545
  Synthetic Polynucleotide

SEQ ID NO: 730 - DNA, 30 bp, Artificial; identical to SEQ ID NO: 546
  Synthetic Polynucleotide

SEQ ID NO: 731 - DNA, 32 bp, Artificial; identical to SEQ ID NO: 547
  Synthetic Polynucleotide

SEQ ID NO: 732 - DNA, 32 bp, Artificial; identical to SEQ ID NO: 548
  Synthetic Polynucleotide

SEQ ID NO: 733 - DNA, 32 bp, Artificial; identical to SEQ ID NO: 549
  Synthetic Polynucleotide

SEQ ID NO: 734 - DNA, 30 bp, Artificial; identical to SEQ ID NO: 550
  Synthetic Polynucleotide

SEQ ID NO: 735 - DNA, 32 bp, Artificial; identical to SEQ ID NO: 551
  Synthetic Polynucleotide

SEQ ID NO: 736 - DNA, 32 bp, Artificial; identical to SEQ ID NO: 552
  Synthetic Polynucleotide

SEQ ID NO: 737 - DNA, 30 bp, Artificial; identical to SEQ ID NO: 553
  Synthetic Polynucleotide

SEQ ID NO: 738 - DNA, 32 bp, Artificial; identical to SEQ ID NO: 554
  Synthetic Polynucleotide

SEQ ID NO: 739 - DNA, 32 bp, Artificial; identical to SEQ ID NO: 555
  Synthetic Polynucleotide

SEQ ID NO: 740 - DNA, 32 bp, Artificial; identical to SEQ ID NO: 556
  Synthetic Polynucleotide

SEQ ID NO: 741 - DNA, 30 bp, Artificial; identical to SEQ ID NO: 557
  Synthetic Polynucleotide

SEQ ID NO: 742 - DNA, 30 bp, Artificial; identical to SEQ ID NO: 558
  Synthetic Polynucleotide

SEQ ID NO: 743 - DNA, 32 bp, Artificial; identical to SEQ ID NO: 559
  Synthetic Polynucleotide

SEQ ID NO: 744 - DNA, 32 bp, Artificial; identical to SEQ ID NO: 560
  Synthetic Polynucleotide

SEQ ID NO: 745 - DNA, 32 bp, Artificial; identical to SEQ ID NO: 561
  Synthetic Polynucleotide

SEQ ID NO: 746 - DNA, 30 bp, Artificial; identical to SEQ ID NO: 562
  Synthetic Polynucleotide

SEQ ID NO: 747 - DNA, 32 bp, Artificial; identical to SEQ ID NO: 563
  Synthetic Polynucleotide

SEQ ID NO: 748 - DNA, 32 bp, Artificial; identical to SEQ ID NO: 564
  Synthetic Polynucleotide

SEQ ID NO: 749 - DNA, 32 bp, Artificial; identical to SEQ ID NO: 565
  Synthetic Polynucleotide

SEQ ID NO: 750 - DNA, 30 bp, Artificial; identical to SEQ ID NO: 566
  Synthetic Polynucleotide

SEQ ID NO: 751 - DNA, 30 bp, Artificial; identical to SEQ ID NO: 567
  Synthetic Polynucleotide

SEQ ID NO: 752 - DNA, 32 bp, Artificial; identical to SEQ ID NO: 568
  Synthetic Polynucleotide

SEQ ID NO: 753 - DNA, 32 bp, Artificial; identical to SEQ ID NO: 569
  Synthetic Polynucleotide

SEQ ID NO: 754 - DNA, 32 bp, Artificial; identical to SEQ ID NO: 570
  Synthetic Polynucleotide

SEQ ID NO: 755 - DNA, 30 bp, Artificial; identical to SEQ ID NO: 571
  Synthetic Polynucleotide

SEQ ID NO: 756 - DNA, 32 bp, Artificial; identical to SEQ ID NO: 572
  Synthetic Polynucleotide

SEQ ID NO: 757 - DNA, 32 bp, Artificial; identical to SEQ ID NO: 573
  Synthetic Polynucleotide

SEQ ID NO: 758 - DNA, 32 bp, Artificial; identical to SEQ ID NO: 574
  Synthetic Polynucleotide

SEQ ID NO: 759 - DNA, 30 bp, Artificial; identical to SEQ ID NO: 575
  Synthetic Polynucleotide

SEQ ID NO: 760 - DNA, 38 bp, Artificial; identical to SEQ ID NO: 576
  Synthetic Polynucleotide

SEQ ID NO: 761 - DNA, 40 bp, Artificial; identical to SEQ ID NO: 577
  Synthetic Polynucleotide

SEQ ID NO: 762 - DNA, 30 bp, Artificial; identical to SEQ ID NO: 578
  Synthetic Polynucleotide

SEQ ID NO: 763 - DNA, 40 bp, Artificial; identical to SEQ ID NO: 579
  Synthetic Polynucleotide

SEQ ID NO: 764 - DNA, 40 bp, Artificial; identical to SEQ ID NO: 580
  Synthetic Polynucleotide

SEQ ID NO: 765 - DNA, 32 bp, Artificial; identical to SEQ ID NO: 581
  Synthetic Polynucleotide

SEQ ID NO: 766 - DNA, 32 bp, Artificial; identical to SEQ ID NO: 582
  Synthetic Polynucleotide

SEQ ID NO: 767 - DNA, 32 bp, Artificial; identical to SEQ ID NO: 583
  Synthetic Polynucleotide

SEQ ID NO: 768 - DNA, 30 bp, Artificial; identical to SEQ ID NO: 584
  Synthetic Polynucleotide

SEQ ID NO: 769 - DNA, 32 bp, Artificial; identical to SEQ ID NO: 585
  Synthetic Polynucleotide

SEQ ID NO: 770 - DNA, 32 bp, Artificial; identical to SEQ ID NO: 586
  Synthetic Polynucleotide

SEQ ID NO: 771 - DNA, 32 bp, Artificial; identical to SEQ ID NO: 587
  Synthetic Polynucleotide

SEQ ID NO: 772 - DNA, 30 bp, Artificial; identical to SEQ ID NO: 588
  Synthetic Polynucleotide

SEQ ID NO: 773 - DNA, 30 bp, Artificial; identical to SEQ ID NO: 589
  Synthetic Polynucleotide

SEQ ID NO: 774 - DNA, 32 bp, Artificial; identical to SEQ ID NO: 590
  Synthetic Polynucleotide

SEQ ID NO: 775 - DNA, 30 bp, Artificial; identical to SEQ ID NO: 591
  Synthetic Polynucleotide

SEQ ID NO: 776 - DNA, 32 bp, Artificial; identical to SEQ ID NO: 592
  Synthetic Polynucleotide

SEQ ID NO: 777 - DNA, 32 bp, Artificial; identical to SEQ ID NO: 593
  Synthetic Polynucleotide

SEQ ID NO: 778 - DNA, 32 bp, Artificial; identical to SEQ ID NO: 594
  Synthetic Polynucleotide

SEQ ID NO: 779 - DNA, 40 bp, Artificial
  Synthetic Polynucleotide
tcatcaaggaacgagtagtaaattcagttgagatttagga

SEQ ID NO: 780 - DNA, 40 bp, Artificial
  Synthetic Polynucleotide
caccagaaggaaccagagccaccaattagagccagcaaaa

SEQ ID NO: 781 - DNA, 40 bp, Artificial
  Synthetic Polynucleotide
ggccttgaatcggcattttcggtcgaaaccatcgatagca

SEQ ID NO: 782 - DNA, 38 bp, Artificial
  Synthetic Polynucleotide
tgaccaacatgcgattttaagaagaaaaatctacgtta

SEQ ID NO: 783 - DNA, 40 bp, Artificial
  Synthetic Polynucleotide
ggtcgacttacgagccggaagcattggtttttcttttcac

SEQ ID NO: 784 - DNA, 40 bp, Artificial
  Synthetic Polynucleotide
ctgagcaatcgggagaaacaataaggagcggaattatcat

SEQ ID NO: 785 - DNA, 40 bp, Artificial
  Synthetic Polynucleotide
catttgaaaagaaattgcgtagatttgtttggattatact

SEQ ID NO: 786 - DNA, 38 bp, Artificial
  Synthetic Polynucleotide
gccagggtttgcgttgcgctcaccagctgcattaatga

SEQ ID NO: 787 - DNA, 43 bp, Artificial
  Synthetic Polynucleotide
acggctacaaaaggagcctttaatgtgagaatttatacatcta

SEQ ID NO: 788 - DNA, 41 bp, Artificial
  Synthetic Polynucleotide
cagcgaaacttgctttcgaggtgttgctaattatacatcta

SEQ ID NO: 789 - DNA, 43 bp, Artificial
  Synthetic Polynucleotide
aaggccgctgataccgatagttgcgacgttagttatacatcta

SEQ ID NO: 790 - DNA, 43 bp, Artificial
  Synthetic Polynucleotide
atattcggaaccatcgcccacgcagagaaggattatacatcta

SEQ ID NO: 791 - DNA, 41 bp, Artificial
  Synthetic Polynucleotide
tattaagaagcggggttttgctcgtagcatttatacatcta

SEQ ID NO: 792 - DNA, 43 bp, Artificial
  Synthetic Polynucleotide
tttcggaagtgccgtcgagagggtgagtttcgttatacatcta

SEQ ID NO: 793 - DNA, 43 bp, Artificial
  Synthetic Polynucleotide
gcccgtatccggaataggtgtatcagcccaatttatacatcta

SEQ ID NO: 794 - DNA, 43 bp, Artificial
  Synthetic Polynucleotide
tacgttaaagtaatcttgacaagaaccgaactttatacatcta

SEQ ID NO: 795 - DNA, 43 bp, Artificial
  Synthetic Polynucleotide
gaaattattgcctttagcgtcagaccggaaccttatacatcta

SEQ ID NO: 796 - DNA, 43 bp, Artificial
  Synthetic Polynucleotide
ctgtagcttgactattatagtcagttcattgattatacatcta

SEQ ID NO: 797 - DNA, 43 bp, Artificial
  Synthetic Polynucleotide
gccagttagagggtaattgagcgctttaagaattatacatcta

SEQ ID NO: 798 - DNA, 43 bp, Artificial
  Synthetic Polynucleotide
aacaagagggataaaaatttttagcataaagcttatacatcta

SEQ ID NO: 799 - DNA, 43 bp, Artificial
  Synthetic Polynucleotide
agtataaagttcagctaatgcagatgtctttcttatacatcta

SEQ ID NO: 800 - DNA, 43 bp, Artificial
  Synthetic Polynucleotide
ccagggttgccagtttgaggggacccgtgggattatacatcta

SEQ ID NO: 801 - DNA, 43 bp, Artificial
  Synthetic Polynucleotide
cctgattgcaatatatgtgagtgatcaatagtttatacatcta

SEQ ID NO: 802 - DNA, 43 bp, Artificial
  Synthetic Polynucleotide
ctccaacgcagtgagacgggcaaccagctgcattatacatcta

SEQ ID NO: 803 - DNA, 41 bp, Artificial
  Synthetic Polynucleotide
tggaacaaccgcctggccctgaggcccgctttatacatcta

SEQ ID NO: 804 - DNA, 43 bp, Artificial
  Synthetic Polynucleotide
gcccgagagtccacgctggtttgcagctaactttatacatcta

SEQ ID NO: 805 - DNA, 43 bp, Artificial
  Synthetic Polynucleotide
tcggcaaatcctgtttgatggtggaccctcaattatacatcta

SEQ ID NO: 806 - DNA, 41 bp, Artificial
  Synthetic Polynucleotide
accttgcttggtcagttggcaaagagcggattatacatcta

SEQ ID NO: 807 - DNA, 43 bp, Artificial
  Synthetic Polynucleotide
agccagcaattgaggaaggttatcatcattttttatacatcta

SEQ ID NO: 808 - DNA, 43 bp, Artificial
  Synthetic Polynucleotide
ttaacaccagcactaacaactaatcgttattattatacatcta

SEQ ID NO: 809 - DNA, 43 bp, Artificial
  Synthetic Polynucleotide
cggattgcagagcttaattgctgaaacgagtattatctacata

SEQ ID NO: 810 - DNA, 43 bp, Artificial
  Synthetic Polynucleotide
cgaaagactttgataagaggtcatatttcgcattatctacata

SEQ ID NO: 811 - DNA, 41 bp, Artificial
  Synthetic Polynucleotide
gcttcaatcaggattagagagttattttcattatctacata

SEQ ID NO: 812 - DNA, 43 bp, Artificial
  Synthetic Polynucleotide
ttagacggccaaataagaaacgatagaaggctttatctacata

SEQ ID NO: 813 - DNA, 41 bp, Artificial
  Synthetic Polynucleotide
aaagtcacaaaataaacagccagcgttttattatctacata

SEQ ID NO: 814 - DNA, 43 bp, Artificial
  Synthetic Polynucleotide
gagagatagagcgtctttccagaggttttgaattatctacata

SEQ ID NO: 815 - DNA, 43 bp, Artificial
  Synthetic Polynucleotide
gatttagtcaataaagcctcagagaaccctcattatctacata

SEQ ID NO: 816 - DNA, 43 bp, Artificial
  Synthetic Polynucleotide
aatggtcaacaggcaaggcaaagagtaatgtgttatctacata

SEQ ID NO: 817 - DNA, 41 bp, Artificial
  Synthetic Polynucleotide
tttggggatagtagtagcattaaaaggccgttatctacata

SEQ ID NO: 818 - DNA, 43 bp, Artificial
  Synthetic Polynucleotide
ccaatagctcatcgtaggaatcatggcatcaattatctacata

SEQ ID NO: 819 - DNA, 43 bp, Artificial
  Synthetic Polynucleotide
tatccggtctcatcgagaacaagcgacaaaagttatctacata

SEQ ID NO: 820 - DNA, 41 bp, Artificial
  Synthetic Polynucleotide
gcgaacctccaagaacgggtatgacaataattatctacata

SEQ ID NO: 821 - DNA, 43 bp, Artificial
  Synthetic Polynucleotide
gccttaaaccaatcaataatcggcacgcgcctttatctacata

SEQ ID NO: 822 - DNA, 43 bp, Artificial
  Synthetic Polynucleotide
taaatcgggattcccaattctgcgatataatgttatctacata

SEQ ID NO: 823 - DNA, 41 bp, Artificial
  Synthetic Polynucleotide
aaattaagttgaccattagatacttttgcgttatctacata

SEQ ID NO: 824 - DNA, 43 bp, Artificial
  Synthetic Polynucleotide
taaatcatataacctgtttagctaacctttaattatctacata

SEQ ID NO: 825 - DNA, 41 bp, Artificial
  Synthetic Polynucleotide
ttttatttaagcaaatcagatattttttgtttatctacata

SEQ ID NO: 826 - DNA, 43 bp, Artificial
  Synthetic Polynucleotide
gtaccgcaattctaagaacgcgagtattatttttatctacata

SEQ ID NO: 827 - DNA, 43 bp, Artificial
  Synthetic Polynucleotide
cttatcattcccgacttgcgggagcctaatttttatctacata

SEQ ID NO: 828 - DNA, 43 bp, Artificial
  Synthetic Polynucleotide
gtaataagttaggcagaggcatttatgatattttatctacata

SEQ ID NO: 829 - DNA, 41 bp, Artificial
  Synthetic Polynucleotide
gctatcagaaatgcaatgcctgaattagcattatctacata

SEQ ID NO: 830 - DNA, 43 bp, Artificial
  Synthetic Polynucleotide
gagggtaggattcaaaagggtgagacatccaattatctacata

SEQ ID NO: 831 - DNA, 41 bp, Artificial
  Synthetic Polynucleotide
catgtaatagaatataaagtaccaagccgtttatctacata

SEQ ID NO: 832 - DNA, 43 bp, Artificial
  Synthetic Polynucleotide
aattgagaattctgtccagacgactaaaccaattatctacata

SEQ ID NO: 833 - DNA, 43 bp, Artificial
  Synthetic Polynucleotide
tccacagacagccctcatagttagcgtaacgatttcttcatta

SEQ ID NO: 834 - DNA, 43 bp, Artificial
  Synthetic Polynucleotide
tcaccagtacaaactacaacgcctagtaccagtttcttcatta

SEQ ID NO: 835 - DNA, 42 bp, Artificial
  Synthetic Polynucleotide
aggaacccatgtaccgtaacacttgatataatttcttcatta

SEQ ID NO: 836 - DNA, 43 bp, Artificial
  Synthetic Polynucleotide
ccaccctcattttcagggatagcaaccgtacttttcttcatta

SEQ ID NO: 837 - DNA, 41 bp, Artificial
  Synthetic Polynucleotide
aggctccagaggctttgaggacacgggtaatttcttcatta

SEQ ID NO: 838 - DNA, 43 bp, Artificial
  Synthetic Polynucleotide
tcatcgccaacaaagtacaacggacgccagcatttcttcatta

SEQ ID NO: 839 - DNA, 41 bp, Artificial
  Synthetic Polynucleotide
aaatcaccttccagtaagcgtcagtaataatttcttcatta

SEQ ID NO: 840 - DNA, 41 bp, Artificial
  Synthetic Polynucleotide
catcaagtaaaacgaactaacgagttgagatttcttcatta

SEQ ID NO: 841 - DNA, 43 bp, Artificial
  Synthetic Polynucleotide
cttttgcagataaaaaccaaaataaagactcctttcttcatta

SEQ ID NO: 842 - DNA, 41 bp, Artificial
  Synthetic Polynucleotide
aatagctatcaatagaaaattcaacattcatttcttcatta

SEQ ID NO: 843 - DNA, 41 bp, Artificial
  Synthetic Polynucleotide
tttaccccaacatgttttaaatttccatattttcttcatta

SEQ ID NO: 844 - DNA, 43 bp, Artificial
  Synthetic Polynucleotide
ttctactacgcgagctgaaaaggttaccgcgctttcttcatta

SEQ ID NO: 845 - DNA, 41 bp, Artificial
  Synthetic Polynucleotide
tgtagaaatcaagattagttgctcttaccatttcttcatta

SEQ ID NO: 846 - DNA, 41 bp, Artificial
  Synthetic Polynucleotide
aacgcaaaatcgatgaacggtaccggttgatttcttcatta

SEQ ID NO: 847 - DNA, 43 bp, Artificial
  Synthetic Polynucleotide
gccatcaagctcattttttaaccacaaatccatttcttcatta

SEQ ID NO: 848 - DNA, 41 bp, Artificial
  Synthetic Polynucleotide
cttagatttaaggcgttaaataaagcctgttttcttcatta

SEQ ID NO: 849 - DNA, 41 bp, Artificial
  Synthetic Polynucleotide
tgcatctttcccagtcacgacggcctgcagtttcttcatta

SEQ ID NO: 850 - DNA, 43 bp, Artificial
  Synthetic Polynucleotide
aagcctggtacgagccggaagcatagatgatgtttcttcatta

SEQ ID NO: 851 - DNA, 41 bp, Artificial
  Synthetic Polynucleotide
ctcgtattagaaattgcgtagatacagtactttcttcatta

SEQ ID NO: 852 - DNA, 41 bp, Artificial
  Synthetic Polynucleotide
ttttcactcaaagggcgaaaaaccatcacctttcttcatta

SEQ ID NO: 853 - DNA, 51 bp, Artificial
  Synthetic Polynucleotide
agctgattgcccttcagagtccactattaaagggtgccgttttcttcatta

SEQ ID NO: 854 - DNA, 43 bp, Artificial
  Synthetic Polynucleotide
agcaagcgtagggttgagtgttgtagggagcctttcttcatta

SEQ ID NO: 855 - DNA, 49 bp, Artificial
  Synthetic Polynucleotide
cccagcaggcgaaaaatcccttataaatcaagccggcgtttcttcatta

SEQ ID NO: 856 - DNA, 43 bp, Artificial
  Synthetic Polynucleotide
tcaatatcgaacctcaaatatcaattccgaaatttcttcatta

SEQ ID NO: 857 - DNA, 41 bp, Artificial
  Synthetic Polynucleotide
ctttaatgcgcgaactgatagccccaccagtttcttcatta

SEQ ID NO: 858 - DNA, 42 bp, Artificial
  Synthetic Polynucleotide
agaaaggaacaactaaaggaattcaaaaaaattatgaatcta

SEQ ID NO: 859 - DNA, 41 bp, Artificial
  Synthetic Polynucleotide
gttttaacttagtaccgccacccagagccattatgaatcta

SEQ ID NO: 860 - DNA, 41 bp, Artificial
  Synthetic Polynucleotide
aatacgtttgaaagaggacagactgaccttttatgaatcta

SEQ ID NO: 861 - DNA, 43 bp, Artificial
  Synthetic Polynucleotide
gatggtttgaacgagtagtaaatttaccattattatgaatcta

SEQ ID NO: 862 - DNA, 41 bp, Artificial
  Synthetic Polynucleotide
accgattgtcggcattttcggtcataatcattatgaatcta

SEQ ID NO: 863 - DNA, 41 bp, Artificial
  Synthetic Polynucleotide
tttaggacaaatgctttaaacaatcaggtcttatgaatcta

SEQ ID NO: 864 - DNA, 43 bp, Artificial
  Synthetic Polynucleotide
ccaacaggagcgaaccagaccggagcctttacttatgaatcta

SEQ ID NO: 865 - DNA, 41 bp, Artificial
  Synthetic Polynucleotide
acgctaacacccacaagaattgaaaatagcttatgaatcta

SEQ ID NO: 866 - DNA, 41 bp, Artificial
  Synthetic Polynucleotide
aacagttttgtaccaaaaacattttatttcttatgaatcta

SEQ ID NO: 867 - DNA, 43 bp, Artificial
  Synthetic Polynucleotide
caaccgtttcaaatcaccatcaattcgagccattatgaatcta

SEQ ID NO: 868 - DNA, 41 bp, Artificial
  Synthetic Polynucleotide
ttagtatcacaatagataagtccacgagcattatgaatcta

SEQ ID NO: 869 - DNA, 41 bp, Artificial
  Synthetic Polynucleotide
taatcagcggattgaccgtaatcgtaaccgttatgaatcta

SEQ ID NO: 870 - DNA, 43 bp, Artificial
  Synthetic Polynucleotide
caactgttgcgccattcgccattcaaacatcattatgaatcta

SEQ ID NO: 871 - DNA, 41 bp, Artificial
  Synthetic Polynucleotide
cttttacaaaatcgtcgctattagcgatagttatgaatcta

SEQ ID NO: 872 - DNA, 41 bp, Artificial
  Synthetic Polynucleotide
gtcgacttcggccaacgcgcggggtttttcttatgaatcta

SEQ ID NO: 873 - DNA, 43 bp, Artificial
  Synthetic Polynucleotide
gcaattcacatattcctgattatcaaagtgtattatgaatcta

SEQ ID NO: 874 - DNA, 41 bp, Artificial
  Synthetic Polynucleotide
cagaagattagataatacatttgtcgacaattatgaatcta

SEQ ID NO: 875 - DNA, 42 bp, Artificial
  Synthetic Polynucleotide
caaatcaagttttttggggtcgaaacgtggattatgaatcta

SEQ ID NO: 876 - DNA, 41 bp, Artificial
  Synthetic Polynucleotide
aaagcactaaatcggaaccctaatccagttttatgaatcta

SEQ ID NO: 877 - DNA, 43 bp, Artificial
  Synthetic Polynucleotide
cccgatttagagcttgacggggaaaaagaatattatgaatcta

SEQ ID NO: 878 - DNA, 42 bp, Artificial
  Synthetic Polynucleotide
aacgtggcgagaaaggaagggaaaccagtaattatgaatcta

SEQ ID NO: 879 - DNA, 41 bp, Artificial
  Synthetic Polynucleotide
taaaagggacattctggccaacaaagcatcttatgaatcta

SEQ ID NO: 880 - DNA, 43 bp, Artificial
  Synthetic Polynucleotide
acccttctgacctgaaagcgtaagacgctgagttatgaatcta

SEQ ID NO: 881 - DNA, 42 bp, Artificial
  Synthetic Polynucleotide
gcacagacaatatttttgaatggggtcagtattatgaatcta

SEQ ID NO: 882 - DNA, 8064 bp, Artificial
  p8064 scaffold sequence for microtubule-like DNA origami structure
tgatagacggtttttcgccctttgacgttggagtccacgttctttaatagtggactcttgttccaaactggaacaacactcaaccctatctcgggctattcttttgatttataagggattttgccgatttcggaaccaccatcaaacaggattttcgcctgctggggcaaaccagcgtggaccgcttgctgcaactctctcagggccaggcggtgaagggcaatcagctgttgcccgtctcactggtgaaaagaaaaaccaccctggcgcccaatacgcaaaccgcctctccccgcgcgttggccgattcattaatgcagctggcacgacaggtttcccgactggaaagcgggcagtgagcgcaacgcaattaatgtgagttagctcactcattaggcaccccaggctttacactttatgcttccggctcgtatgttgtgtggaattgtgagcggataacaatttcacacaggaaacagctatgaccatgattacgaattcgagctcggtacccggggatcctcaactgtgaggaggctcacggacgcgaagaacaggcacgcgtgctggcagaaacccccggtatgaccgtgaaaacggcccgccgcattctggccgcagcaccacagagtgcacaggcgcgcagtgacactgcgctggatcgtctgatgcagggggcaccggcaccgctggctgcaggtaacccggcatctgatgccgttaacgatttgctgaacacaccagtgtaagggatgtttatgacgagcaaagaaacctttacccattaccagccgcagggcaacagtgacccggctcataccgcaaccgcgcccggcggattgagtgcgaaagcgcctgcaatgaccccgctgatgctggacacctccagccgtaagctggttgcgtgggatggcaccaccgacggtgctgccgttggcattcttgcggttgctgctgaccagaccagcaccacgctgacgttctacaagtccggcacgttccgttatgaggatgtgctctggccggaggctgccagcgacgagacgaaaaaacggaccgcgtttgccggaacggcaatcagcatcgtttaactttacccttcatcactaaaggccgcctgtgcggctttttttacgggatttttttatgtcgatgtacacaaccgcccaactgctggcggcaaatgagcagaaatttaagtttgatccgctgtttctgcgtctctttttccgtgagagctatcccttcaccacggagaaagtctatctctcacaaattccgggactggtaaacatggcgctgtacgtttcgccgattgtttccggtgaggttatccgttcccgtggcggctccacctctgaaagcttggcactggccgtcgttttacaacgtcgtgactgggaaaaccctggcgttacccaacttaatcgccttgcagcacatccccctttcgccagctggcgtaatagcgaagaggcccgcaccgatcgcccttcccaacagttgcgcagcctgaatggcgaatggcgctttgcctggtttccggcaccagaagcggtgccggaaagctggctggagtgcgatcttcctgaggccgatactgtcgtcgtcccctcaaactggcagatgcacggttacgatgcgcccatctacaccaacgtgacctatcccattacggtcaatccgccgtttgttcccacggagaatccgacgggttgttactcgctcacatttaatgttgatgaaagctggctacaggaaggccagacgcgaattatttttgatggcgttcctattggttaaaaaatgagctgatttaacaaaaatttaatgcgaattttaacaaaatattaacgtttacaatttaaatatttgcttatacaatcttcctgtttttggggcttttctgattatcaaccggggtacatatgattgacatgctagttttacgattaccgttcatcgattctcttgtttgctccagactctcaggcaatgacctgatagcctttgtagatctctcaaaaatagctaccctctccggcattaatttatcagctagaacggttgaatatcatattgatggtgatttgactgtctccggcctttctcacccttttgaatctttacctacacattactcaggcattgcatttaaaatatatgagggttctaaaaatttttatccttgcgttgaaataaaggcttctcccgcaaaagtattacagggtcataatgtttttggtacaaccgatttagctttatgctctgaggctttattgcttaattttgctaattctttgccttgcctgtatgatttattggatgttaatgctactactattagtagaattgatgccaccttttcagctcgcgccccaaatgaaaatatagctaaacaggttattgaccatttgcgaaatgtatctaatggtcaaactaaatctactcgttcgcagaattgggaatcaactgttatatggaatgaaacttccagacaccgtactttagttgcatatttaaaacatgttgagctacagcattatattcagcaattaagctctaagccatccgcaaaaatgacctcttatcaaaaggagcaattaaaggtactctctaatcctgacctgttggagtttgcttccggtctggttcgctttgaagctcgaattaaaacgcgatatttgaagtctttcgggcttcctcttaatctttttgatgcaatccgctttgcttctgactataatagtcagggtaaagacctgatttttgatttatggtcattctcgttttctgaactgtttaaagcatttgagggggattcaatgaatatttatgacgattccgcagtattggacgctatccagtctaaacattttactattaccccctctggcaaaacttcttttgcaaaagcctctcgctattttggtttttatcgtcgtctggtaaacgagggttatgatagtgttgctcttactatgcctcgtaattccttttggcgttatgtatctgcattagttgaatgtggtattcctaaatctcaactgatgaatctttctacctgtaataatgttgttccgttagttcgttttattaacgtagatttttcttcccaacgtcctgactggtataatgagccagttcttaaaatcgcataaggtaattcacaatgattaaagttgaaattaaaccatctcaagcccaatttactactcgttctggtgtttctcgtcagggcaagccttattcactgaatgagcagctttgttacgttgatttgggtaatgaatatccggttcttgtcaagattactcttgatgaaggtcagccagcctatgcgcctggtctgtacaccgttcatctgtcctctttcaaagttggtcagttcggttcccttatgattgaccgtctgcgcctcgttccggctaagtaacatggagcaggtcgcggatttcgacacaatttatcaggcgatgatacaaatctccgttgtactttgtttcgcgcttggtataatcgctgggggtcaaagatgagtgttttagtgtattcttttgcctctttcgttttaggttggtgccttcgtagtggcattacgtattttacccgtttaatggaaacttcctcatgaaaaagtctttagtcctcaaagcctctgtagccgttgctaccctcgttccgatgctgtctttcgctgctgagggtgacgatcccgcaaaagcggcctttaactccctgcaagcctcagcgaccgaatatatcggttatgcgtgggcgatggttgttgtcattgtcggcgcaactatcggtatcaagctgtttaagaaattcacctcgaaagcaagctgataaaccgatacaattaaaggctccttttggagccttttttttggagattttcaacgtgaaaaaattattattcgcaattcctttagttgttcctttctattctcactccgctgaaactgttgaaagttgtttagcaaaatcccatacagaaaattcatttactaacgtctggaaagacgacaaaactttagatcgttacgctaactatgagggctgtctgtggaatgctacaggcgttgtagtttgtactggtgacgaaactcagtgttacggtacatgggttcctattgggcttgctatccctgaaaatgagggtggtggctctgagggtggcggttctgagggtggcggttctgagggtggcggtactaaacctcctgagtacggtgatacacctattccgggctatacttatatcaaccctctcgacggcacttatccgcctggtactgagcaaaaccccgctaatcctaatccttctcttgaggagtctcagcctcttaatactttcatgtttcagaataataggttccgaaataggcagggggcattaactgtttatacgggcactgttactcaaggcactgaccccgttaaaacttattaccagtacactcctgtatcatcaaaagccatgtatgacgcttactggaacggtaaattcagagactgcgctttccattctggctttaatgaggatttatttgtttgtgaatatcaaggccaatcgtctgacctgcctcaacctcctgtcaatgctggcggcggctctggtggtggttctggtggcggctctgagggtggtggctctgagggtggcggttctgagggtggcggctctgagggaggcggttccggtggtggctctggttccggtgattttgattatgaaaagatggcaaacgctaataagggggctatgaccgaaaatgccgatgaaaacgcgctacagtctgacgctaaaggcaaacttgattctgtcgctactgattacggtgctgctatcgatggtttcattggtgacgtttccggccttgctaatggtaatggtgctactggtgattttgctggctctaattcccaaatggctcaagtcggtgacggtgataattcacctttaatgaataatttccgtcaatatttaccttccctccctcaatcggttgaatgtcgcccttttgtctttggcgctggtaaaccatatgaattttctattgattgtgacaaaataaacttattccgtggtgtctttgcgtttcttttatatgttgccacctttatgtatgtattttctacgtttgctaacatactgcgtaataaggagtcttaatcatgccagttcttttgggtattccgttattattgcgtttcctcggtttccttctggtaactttgttcggctatctgcttacttttcttaaaaagggcttcggtaagatagctattgctatttcattgtttcttgctcttattattgggcttaactcaattcttgtgggttatctctctgatattagcgctcaattaccctctgactttgttcagggtgttcagttaattctcccgtctaatgcgcttccctgtttttatgttattctctctgtaaaggctgctattttcatttttgacgttaaacaaaaaatcgtttcttatttggattgggataaataatatggctgtttattttgtaactggcaaattaggctctggaaagacgctcgttagcgttggtaagattcaggataaaattgtagctgggtgcaaaatagcaactaatcttgatttaaggcttcaaaacctcccgcaagtcgggaggttcgctaaaacgcctcgcgttcttagaataccggataagccttctatatctgatttgcttgctattgggcgcggtaatgattcctacgatgaaaataaaaacggcttgcttgttctcgatgagtgcggtacttggtttaatacccgttcttggaatgataaggaaagacagccgattattgattggtttctacatgctcgtaaattaggatgggatattatttttcttgttcaggacttatctattgttgataaacaggcgcgttctgcattagctgaacatgttgtttattgtcgtcgtctggacagaattactttaccttttgtcggtactttatattctcttattactggctcgaaaatgcctctgcctaaattacatgttggcgttgttaaatatggcgattctcaattaagccctactgttgagcgttggctttatactggtaagaatttgtataacgcatatgatactaaacaggctttttctagtaattatgattccggtgtttattcttatttaacgccttatttatcacacggtcggtatttcaaaccattaaatttaggtcagaagatgaaattaactaaaatatatttgaaaaagttttctcgcgttctttgtcttgcgattggatttgcatcagcatttacatatagttatataacccaacctaagccggaggttaaaaaggtagtctctcagacctatgattttgataaattcactattgactcttctcagcgtcttaatctaagctatcgctatgttttcaaggattctaagggaaaattaattaatagcgacgatttacagaagcaaggttattcactcacatatattgatttatgtactgtttccattaaaaaaggtaattcaaatgaaattgttaaatgtaattaattttgttttcttgatgtttgtttcatcatcttcttttgctcaggtaattgaaatgaataattcgcctctgcgcgattttgtaacttggtattcaaagcaatcaggcgaatccgttattgtttctcccgatgtaaaaggtactgttactgtatattcatctgacgttaaacctgaaaatctacgcaatttctttatttctgttttacgtgcaaataattttgatatggtaggttctaacccttccattattcagaagtataatccaaacaatcaggattatattgatgaattgccatcatctgataatcaggaatatgatgataattccgctccttctggtggtttctttgttccgcaaaatgataatgttactcaaacttttaaaattaataacgttcgggcaaaggatttaatacgagttgtcgaattgtttgtaaagtctaatacttctaaatcctcaaatgtattatctattgacggctctaatctattagttgttagtgctcctaaagatattttagataaccttcctcaattcctttcaactgttgatttgccaactgaccagatattgattgagggtttgatatttgaggttcagcaaggtgatgctttagatttttcatttgctgctggctctcagcgtggcactgttgcaggcggtgttaatactgaccgcctcacctctgttttatcttctgctggtggttcgttcggtatttttaatggcgatgttttagggctatcagttcgcgcattaaagactaatagccattcaaaaatattgtctgtgccacgtattcttacgctttcaggtcagaagggttctatctctgttggccagaatgtcccttttattactggtcgtgtgactggtgaatctgccaatgtaaataatccatttcagacgattgagcgtcaaaatgtaggtatttccatgagcgtttttcctgttgcaatggctggcggtaatattgttctggatattaccagcaaggccgatagtttgagttcttctactcaggcaagtgatgttattactaatcaaagaagtattgctacaacggttaatttgcgtgatggacagactcttttactcggtggcctcactgattataaaaacacttctcaggattctggcgtaccgttcctgtctaaaatccctttaatcggcctcctgtttagctcccgctctgattctaacgaggaaagcacgttatacgtgctcgtcaaagcaaccatagtacgcgccctgtagcggcgcattaagcgcggcgggtgtggtggttacgcgcagcgtgaccgctacacttgccagcgccctagcgcccgctcctttcgctttcttcccttcctttctcgccacgttcgccggctttccccgtcaagctctaaatcgggggctccctttagggttccgatttagtgctttacggcacctcgaccccaaaaaacttgatttgggtgatggttcacgtagtgggccatcgccc

SEQ ID NO: 883 - DNA, 6912 bp, Artificial
  M13mp18 scaffold sequence for drift markers and Exchange-PAINT DNAorigami structures
ttcccttcctttctcgccacgttcgccggctttccccgtcaagctctaaatcgggggctccctttagggttccgatttagtgctttacggcacctcgaccccaaaaaacttgatttgggtgatggttcacgtagtgggccatcgccctgatagacggtttttcgccctttgacgttggagtccacgttctttaatagtggactcttgttccaaactggaacaacactcaaccctatctcgggctattcttttgatttataagggattttgccgatttcggaaccaccatcaaacaggattttcgcctgctggggcaaaccagcgtggaccgcttgctgcaactctctcagggccaggcggtgaagggcaatcagctgttgcccgtctcactggtgaaaagaaaaaccaccctggcgcccaatacgcaaaccgcctctccccgcgcgttggccgattcattaatgcagctggcacgacaggtttcccgactggaaagcgggcagtgagcgcaacgcaattaatgtgagttagctcactcattaggcaccccaggctttacactttatgcttccggctcgtatgttgtgtggaattgtgagcggataacaatttcacacaggaaacagctatgaccatgattacgaattcgagctcggtacccggggatcctctagagtcgacctgcaggcatgcaagcttggcactggccgtcgttttacaacgtcgtgactgggaaaaccctggcgttacccaacttaatcgccttgcagcacatccccctttcgccagctggcgtaatagcgaagaggcccgcaccgatcgcccttcccaacagttgcgcagcctgaatggcgaatggcgctttgcctggtttccggcaccagaagcggtgccggaaagctggctggagtgcgatcttcctgaggccgatactgtcgtcgtcccctcaaactggcagatgcacggttacgatgcgcccatctacaccaacgtgacctatcccattacggtcaatccgccgtttgttcccacggagaatccgacgggttgttactcgctcacatttaatgttgatgaaagctggctacaggaaggccagacgcgaattatttttgatggcgttcctattggttaaaaaatgagctgatttaacaaaaatttaatgcgaattttaacaaaatattaacgtttacaatttaaatatttgcttatacaatcttcctgtttttggggcttttctgattatcaaccggggtacatatgattgacatgctagttttacgattaccgttcatcgattctcttgtttgctccagactctcaggcaatgacctgatagcctttgtagatctctcaaaaatagctaccctctccggcattaatttatcagctagaacggttgaatatcatattgatggtgatttgactgtctccggcctttctcacccttttgaatctttacctacacattactcaggcattgcatttaaaatatatgagggttctaaaaatttttatccttgcgttgaaataaaggcttctcccgcaaaagtattacagggtcataatgtttttggtacaaccgatttagctttatgctctgaggctttattgcttaattttgctaattctttgccttgcctgtatgatttattggatgttaatgctactactattagtagaattgatgccaccttttcagctcgcgccccaaatgaaaatatagctaaacaggttattgaccatttgcgaaatgtatctaatggtcaaactaaatctactcgttcgcagaattgggaatcaactgttatatggaatgaaacttccagacaccgtactttagttgcatatttaaaacatgttgagctacagcattatattcagcaattaagctctaagccatccgcaaaaatgacctcttatcaaaaggagcaattaaaggtactctctaatcctgacctgttggagtttgcttccggtctggttcgctttgaagctcgaattaaaacgcgatatttgaagtctttcgggcttcctcttaatctttttgatgcaatccgctttgcttctgactataatagtcagggtaaagacctgatttttgatttatggtcattctcgttttctgaactgtttaaagcatttgagggggattcaatgaatatttatgacgattccgcagtattggacgctatccagtctaaacattttactattaccccctctggcaaaacttcttttgcaaaagcctctcgctattttggtttttatcgtcgtctggtaaacgagggttatgatagtgttgctcttactatgcctcgtaattccttttggcgttatgtatctgcattagttgaatgtggtattcctaaatctcaactgatgaatctttctacctgtaataatgttgttccgttagttcgttttattaacgtagatttttcttcccaacgtcctgactggtataatgagccagttcttaaaatcgcataaggtaattcacaatgattaaagttgaaattaaaccatctcaagcccaatttactactcgttctggtgtttctcgtcagggcaagccttattcactgaatgagcagctttgttacgttgatttgggtaatgaatatccggttcttgtcaagattactcttgatgaaggtcagccagcctatgcgcctggtctgtacaccgttcatctgtcctctttcaaagttggtcagttcggttcccttatgattgaccgtctgcgcctcgttccggctaagtaacatggagcaggtcgcggatttcgacacaatttatcaggcgatgatacaaatctccgttgtactttgtttcgcgcttggtataatcgctgggggtcaaagatgagtgttttagtgtattcttttgcctctttcgttttaggttggtgccttcgtagtggcattacgtattttacccgtttaatggaaacttcctcatgaaaaagtctttagtcctcaaagcctctgtagccgttgctaccctcgttccgatgctgtctttcgctgctgagggtgacgatcccgcaaaagcggcctttaactccctgcaagcctcagcgaccgaatatatcggttatgcgtgggcgatggttgttgtcattgtcggcgcaactatcggtatcaagctgtttaagaaattcacctcgaaagcaagctgataaaccgatacaattaaaggctccttttggagccttttttttggagattttcaacgtgaaaaaattattattcgcaattcctttagttgttcctttctattctcactccgctgaaactgttgaaagttgtttagcaaaatcccatacagaaaattcatttactaacgtctggaaagacgacaaaactttagatcgttacgctaactatgagggctgtctgtggaatgctacaggcgttgtagtttgtactggtgacgaaactcagtgttacggtacatgggttcctattgggcttgctatccctgaaaatgagggtggtggctctgagggtggcggttctgagggtggcggttctgagggtggcggtactaaacctcctgagtacggtgatacacctattccgggctatacttatatcaaccctctcgacggcacttatccgcctggtactgagcaaaaccccgctaatcctaatccttctcttgaggagtctcagcctcttaatactttcatgtttcagaataataggttccgaaataggcagggggcattaactgtttatacgggcactgttactcaaggcactgaccccgttaaaacttattaccagtacactcctgtatcatcaaaagccatgtatgacgcttactggaacggtaaattcagagactgcgctttccattctggctttaatgaggatttatttgtttgtgaatatcaaggccaatcgtctgacctgcctcaacctcctgtcaatgctggcggcggctctggtggtggttctggtggcggctctgagggtggtggctctgagggtggcggttctgagggtggcggctctgagggaggcggttccggtggtggctctggttccggtgattttgattatgaaaagatggcaaacgctaataagggggctatgaccgaaaatgccgatgaaaacgcgctacagtctgacgctaaaggcaaacttgattctgtcgctactgattacggtgctgctatcgatggtttcattggtgacgtttccggccttgctaatggtaatggtgctactggtgattttgctggctctaattcccaaatggctcaagtcggtgacggtgataattcacctttaatgaataatttccgtcaatatttaccttccctccctcaatcggttgaatgtcgcccttttgtctttggcgctggtaaaccatatgaattttctattgattgtgacaaaataaacttattccgtggtgtctttgcgtttcttttatatgttgccacctttatgtatgtattttctacgtttgctaacatactgcgtaataaggagtcttaatcatgccagttcttttgggtattccgttattattgcgtttcctcggtttccttctggtaactttgttcggctatctgcttacttttcttaaaaagggcttcggtaagatagctattgctatttcattgtttcttgctcttattattgggcttaactcaattcttgtgggttatctctctgatattagcgctcaattaccctctgactttgttcagggtgttcagttaattctcccgtctaatgcgcttccctgtttttatgttattctctctgtaaaggctgctattttcatttttgacgttaaacaaaaaatcgtttcttatttggattgggataaataatatggctgtttattttgtaactggcaaattaggctctggaaagacgctcgttagcgttggtaagattcaggataaaattgtagctgggtgcaaaatagcaactaatcttgatttaaggcttcaaaacctcccgcaagtcgggaggttcgctaaaacgcctcgcgttcttagaataccggataagccttctatatctgatttgcttgctattgggcgcggtaatgattcctacgatgaaaataaaaacggcttgcttgttctcgatgagtgcggtacttggtttaatacccgttcttggaatgataaggaaagacagccgattattgattggtttctacatgctcgtaaattaggatgggatattatttttcttgttcaggacttatctattgttgataaacaggcgcgttctgcattagctgaacatgttgtttattgtcgtcgtctggacagaattactttaccttttgtcggtactttatattctcttattactggctcgaaaatgcctctgcctaaattacatgttggcgttgttaaatatggcgattctcaattaagccctactgttgagcgttggctttatactggtaagaatttgtataacgcatatgatactaaacaggctttttctagtaattatgattccggtgtttattcttatttaacgccttatttatcacacggtcggtatttcaaaccattaaatttaggtcagaagatgaaattaactaaaatatatttgaaaaagttttctcgcgttctttgtcttgcgattggatttgcatcagcatttacatatagttatataacccaacctaagccggaggttaaaaaggtagtctctcagacctatgattttgataaattcactattgactcttctcagcgtcttaatctaagctatcgctatgttttcaaggattctaagggaaaattaattaatagcgacgatttacagaagcaaggttattcactcacatatattgatttatgtactgtttccattaaaaaaggtaattcaaatgaaattgttaaatgtaattaattttgttttcttgatgtttgtttcatcatcttcttttgctcaggtaattgaaatgaataattcgcctctgcgcgattttgtaacttggtattcaaagcaatcaggcgaatccgttattgtttctcccgatgtaaaaggtactgttactgtatattcatctgacgttaaacctgaaaatctacgcaatttctttatttctgttttacgtgcaaataattttgatatggtaggttctaacccttccattattcagaagtataatccaaacaatcaggattatattgatgaattgccatcatctgataatcaggaatatgatgataattccgctccttctggtggtttctttgttccgcaaaatgataatgttactcaaacttttaaaattaataacgttcgggcaaaggatttaatacgagttgtcgaattgtttgtaaagtctaatacttctaaatcctcaaatgtattatctattgacggctctaatctattagttgttagtgctcctaaagatattttagataaccttcctcaattcctttcaactgttgatttgccaactgaccagatattgattgagggtttgatatttgaggttcagcaaggtgatgctttagatttttcatttgctgctggctctcagcgtggcactgttgcaggcggtgttaatactgaccgcctcacctctgttttatcttctgctggtggttcgttcggtatttttaatggcgatgttttagggctatcagttcgcgcattaaagactaatagccattcaaaaatattgtctgtgccacgtattcttacgctttcaggtcagaagggttctatctctgttggccagaatgtcccttttattactggtcgtgtgactggtgaatctgccaatgtaaataatccatttcagacgattgagcgtcaaaatgtaggtatttccatgagcgtttttcctgttgcaatggctggcggtaatattgttctggatattaccagcaaggccgatagtttg

SEQ ID NO: 884 - DNA, 10 bp, Artificial
  Synthetic Polynucleotide
ctagatgtat

SEQ ID NO: 885 - DNA, 10 bp, Artificial
  Synthetic Polynucleotide
tatgtagatc

SEQ ID NO: 886 - DNA, 10 bp, Artificial
  Synthetic Polynucleotide
gtaatgaaga

SEQ ID NO: 887 - DNA, 10 bp, Artificial
  Synthetic Polynucleotide
gtagattcat

SEQ ID NO: 888 - DNA, 10 bp, Artificial
  Synthetic Polynucleotide
ctttacctaa

SEQ ID NO: 889 - DNA, 10 bp, Artificial
  Synthetic Polynucleotide
gtactcaatt

SEQ ID NO: 890 - DNA, 10 bp, Artificial
  Synthetic Polynucleotide
catcctaatt

SEQ ID NO: 891 - DNA, 10 bp, Artificial
  Synthetic Polynucleotide
gatccattat

SEQ ID NO: 892 - DNA, 10 bp, Artificial
  Synthetic Polynucleotide
caccttatta

SEQ ID NO: 893 - DNA, 10 bp, Artificial
  Synthetic Polynucleotide
ccttctctat

SEQ ID NO: 894 - DNA, 10 bp, Artificial
  Synthetic Polynucleotide
gtatcatcaa

SEQ ID NO: 895 - DNA, 10 bp, Artificial
  Synthetic Polynucleotide
gaatcactat

SEQ ID NO: 896 - DNA, 11 bp, Artificial
  Synthetic Polynucleotide
ttatacatcta

SEQ ID NO: 897 - DNA, 11 bp, Artificial
  Synthetic Polynucleotide
ttatctacata

SEQ ID NO: 898 - DNA, 12 bp, Artificial
  Synthetic Polynucleotide
ttgatctacata

SEQ ID NO: 899 - DNA, 11 bp, Artificial
  Synthetic Polynucleotide
tttcttcatta

SEQ ID NO: 900 - DNA, 11 bp, Artificial
  Synthetic Polynucleotide
ttatgaatcta

SEQ ID NO: 901 - DNA, 11 bp, Artificial
  Synthetic Polynucleotide
ttttaggtaaa

SEQ ID NO: 902 - DNA, 11 bp, Artificial
  Synthetic Polynucleotide
ttaattgagta

SEQ ID NO: 903 - DNA, 11 bp, Artificial
  Synthetic Polynucleotide
ttaattaggat

SEQ ID NO: 904 - DNA, 11 bp, Artificial
  Synthetic Polynucleotide
ttataatggat

SEQ ID NO: 905 - DNA, 11 bp, Artificial
  Synthetic Polynucleotide
tttaataaggt

SEQ ID NO: 906 - DNA, 11 bp, Artificial
  Synthetic Polynucleotide
ttatagagaag

SEQ ID NO: 907 - DNA, 11 bp, Artificial
  Synthetic Polynucleotide
ttttgatgata

SEQ ID NO: 908 - DNA, 11 bp, Artificial
  Synthetic Polynucleotide
ttatagtgatt

SEQ ID NO: 909 - DNA, 11 bp, Artificial
  Synthetic Polynucleotide
ttatacatcta

SEQ ID NO: 910 - DNA, 11 bp, Artificial
  Synthetic Polynucleotide
ttatctacata

SEQ ID NO: 911 - DNA, 11 bp, Artificial
  Synthetic Polynucleotide
tttcttcatta

SEQ ID NO: 912 - DNA, 11 bp, Artificial
  Synthetic Polynucleotide
ttatgaatcta

SEQ ID NO: 913 - DNA, 21 bp, Artificial
  Synthetic Polynucleotide
gaatcggtcacagtacaaccg